European Patent Specification EP 3 617 314 B1, published February 15, 2023. Title: nucleotide derivative and salt thereof. Applicant: Kyowa Hakko Kirin Co., Ltd. The sequence listing filed with the application follows.

SEQUENCE LISTING (74 sequences)

SEQ ID NO: 1 - RNA, 21 nt, Artificial Sequence
  HPRT1_ssRNA1
  modified_base (1)..(1): 2'-deoxy-2'-fluoroadenosine
  misc_feature (1)..(2): 5'-phosphorothioated
  modified_base (2)..(2): 2'-methoxyadenosine
  misc_feature (2)..(3): 5'-phosphorothioated
  modified_base (3)..(3): 2'-deoxy-2'-fluoroguanosine
  modified_base (4)..(4): 2'-methoxycytidine
  modified_base (5)..(5): 2'-deoxy-2'-fluorocytidine
  modified_base (6)..(6): 2'-methoxyadenosine
  modified_base (7)..(7): 2'-deoxy-2'-fluoroguanosine
  modified_base (8)..(8): 2'-methoxyadenosine
  modified_base (9)..(9): 2'-deoxy-2'-fluorocytidine
  modified_base (10)..(10): 2'-methoxyuridine
  modified_base (11)..(11): 2'-deoxy-2'-fluorouridine
  modified_base (12)..(12): 2'-methoxyuridine
  modified_base (13)..(13): 2'-deoxy-2'-fluoroguanosine
  modified_base (14)..(14): 2'-methoxyuridine
  modified_base (15)..(15): 2'-deoxy-2'-fluorouridine
  modified_base (16)..(16): 2'-methoxyguanosine
  modified_base (17)..(17): 2'-deoxy-2'-fluoroguanosine
  modified_base (18)..(18): 2'-methoxyadenosine
  modified_base (19)..(19): 2'-deoxy-2'-fluorouridine
  modified_base (20)..(20): 2'-methoxyuridine
  modified_base (21)..(21): 2'-deoxy-2'-fluorouridine
aagccagacuuuguuggauuu

SEQ ID NO: 2 - RNA, 21 nt, Artificial Sequence
  HPRT1_ssRNA2
  modified_base (1)..(1): 2'-deoxy-2'-fluorouridine
  modified_base (2)..(2): 2'-methoxycytidine
  modified_base (3)..(3): 2'-deoxy-2'-fluorocytidine
  modified_base (4)..(4): 2'-methoxyuridine
  modified_base (5)..(5): 2'-deoxy-2'-fluoroadenosine
  modified_base (6)..(6): 2'-methoxyuridine
  modified_base (7)..(7): 2'-deoxy-2'-fluoroguanosine
  modified_base (8)..(8): 2'-methoxyadenosine
  modified_base (9)..(9): 2'-deoxy-2'-fluorocytidine
  modified_base (10)..(10): 2'-methoxyuridine
  modified_base (11)..(11): 2'-deoxy-2'-fluoroguanosine
  modified_base (12)..(12): 2'-methoxyuridine
  modified_base (13)..(13): 2'-deoxy-2'-fluoroadenosine
  modified_base (14)..(14): 2'-methoxyguanosine
  modified_base (15)..(15): 2'-deoxy-2'-fluoroadenosine
  modified_base (16)..(16): 2'-methoxyuridine
  modified_base (17)..(17): 2'-deoxy-2'-fluorouridine
  modified_base (18)..(18): 2'-methoxyuridine
  modified_base (19)..(19): 2'-deoxy-2'-fluorouridine
  modified_base (20)..(20): 2'-methoxyadenosine
  modified_base (21)..(21): 2'-deoxy-2'-fluorouridine
uccuaugacuguagauuuuau

SEQ ID NO: 3 - RNA, 21 nt, Artificial Sequence
  HPRT1_ssRNA3
  modified_base (1)..(1): 2'-deoxy-2'-fluorouridine
  misc_feature (1)..(2): 5'-phosphorothioated
  modified_base (2)..(2): 2'-methoxycytidine
  misc_feature (2)..(3): 5'-phosphorothioated
  modified_base (3)..(3): 2'-deoxy-2'-fluorocytidine
  modified_base (4)..(4): 2'-methoxyuridine
  modified_base (5)..(5): 2'-deoxy-2'-fluoroadenosine
  modified_base (6)..(6): 2'-methoxyuridine
  modified_base (7)..(7): 2'-deoxy-2'-fluoroguanosine
  modified_base (8)..(8): 2'-methoxyadenosine
  modified_base (9)..(9): 2'-deoxy-2'-fluorocytidine
  modified_base (10)..(10): 2'-methoxyuridine
  modified_base (11)..(11): 2'-deoxy-2'-fluoroguanosine
  modified_base (12)..(12): 2'-methoxyuridine
  modified_base (13)..(13): 2'-deoxy-2'-fluoroadenosine
  modified_base (14)..(14): 2'-methoxyguanosine
  modified_base (15)..(15): 2'-deoxy-2'-fluoroadenosine
  modified_base (16)..(16): 2'-methoxyuridine
  modified_base (17)..(17): 2'-deoxy-2'-fluorouridine
  modified_base (18)..(18): 2'-methoxyuridine
  modified_base (19)..(19): 2'-deoxy-2'-fluorouridine
  misc_feature (19)..(20): 5'-phosphorothioated
  modified_base (20)..(20): 2'-methoxyadenosine
  misc_feature (20)..(21): 5'-phosphorothioated
  modified_base (21)..(21): 2'-deoxy-2'-fluorouridine
uccuaugacuguagauuuuau

SEQ ID NO: 4 - RNA, 21 nt, Artificial Sequence
  HPRT1_ssRNA4
  modified_base (1)..(1): 2'-deoxy-2'-fluorouridine
  misc_feature (1)..(2): 5'-phosphorothioated
  modified_base (2)..(2): 2'-methoxycytidine
  misc_feature (2)..(3): 5'-phosphorothioated
  modified_base (3)..(3): 2'-deoxy-2'-fluorocytidine
  misc_feature (3)..(4): 5'-phosphorothioated
  modified_base (4)..(4): 2'-methoxyuridine
  misc_feature (4)..(5): 5'-phosphorothioated
  modified_base (5)..(5): 2'-deoxy-2'-fluoroadenosine
  misc_feature (5)..(6): 5'-phosphorothioated
  modified_base (6)..(6): 2'-methoxyuridine
  misc_feature (6)..(7): 5'-phosphorothioated
  modified_base (7)..(7): 2'-deoxy-2'-fluoroguanosine
  misc_feature (7)..(8): 5'-phosphorothioated
  modified_base (8)..(8): 2'-methoxyadenosine
  modified_base (9)..(9): 2'-deoxy-2'-fluorocytidine
  modified_base (10)..(10): 2'-methoxyuridine
  modified_base (11)..(11): 2'-deoxy-2'-fluoroguanosine
  modified_base (12)..(12): 2'-methoxyuridine
  modified_base (13)..(13): 2'-deoxy-2'-fluoroadenosine
  misc_feature (13)..(14): 5'-phosphorothioated
  modified_base (14)..(14): 2'-methoxyguanosine
  misc_feature (14)..(15): 5'-phosphorothioated
  modified_base (15)..(15): 2'-deoxy-2'-fluoroadenosine
  misc_feature (15)..(16): 5'-phosphorothioated
  modified_base (16)..(16): 2'-methoxyuridine
  misc_feature (16)..(17): 5'-phosphorothioated
  modified_base (17)..(17): 2'-deoxy-2'-fluorouridine
  misc_feature (17)..(18): 5'-phosphorothioated
  modified_base (18)..(18): 2'-methoxyuridine
  misc_feature (18)..(19): 5'-phosphorothioated
  modified_base (19)..(19): 2'-deoxy-2'-fluorouridine
  misc_feature (19)..(20): 5'-phosphorothioated
  modified_base (20)..(20): 2'-methoxyadenosine
  misc_feature (20)..(21): 5'-phosphorothioated
  modified_base (21)..(21): 2'-deoxy-2'-fluorouridine
uccuaugacuguagauuuuau

SEQ ID NO: 5 - RNA, 25 nt, Artificial Sequence
  HPRT1_ssRNA5
  modified_base (1)..(1): 2'-deoxy-2'-fluoroadenosine
  misc_feature (1)..(2): 5'-phosphorothioated
  modified_base (2)..(2): 2'-methoxyuridine
  misc_feature (2)..(3): 5'-phosphorothioated
  modified_base (3)..(3): 2'-deoxy-2'-fluoroadenosine
  modified_base (4)..(4): 2'-methoxyuridine
  modified_base (5)..(5): 2'-deoxy-2'-fluoroadenosine
  modified_base (6)..(6): 2'-methoxyadenosine
  modified_base (7)..(7): 2'-deoxy-2'-fluoroguanosine
  modified_base (8)..(8): 2'-methoxycytidine
  modified_base (9)..(9): 2'-deoxy-2'-fluorocytidine
  modified_base (10)..(10): 2'-methoxyadenosine
  modified_base (11)..(11): 2'-deoxy-2'-fluoroguanosine
  modified_base (12)..(12): 2'-methoxyadenosine
  modified_base (13)..(13): 2'-deoxy-2'-fluorocytidine
  modified_base (14)..(14): 2'-methoxyuridine
  modified_base (15)..(15): 2'-deoxy-2'-fluorouridine
  modified_base (16)..(16): 2'-methoxyuridine
  modified_base (17)..(17): 2'-deoxy-2'-fluoroguanosine
  modified_base (18)..(18): 2'-methoxyuridine
  modified_base (19)..(19): 2'-deoxy-2'-fluorouridine
  modified_base (20)..(20): 2'-methoxyguanosine
  modified_base (21)..(21): 2'-deoxy-2'-fluoroguanosine
  modified_base (22)..(22): 2'-methoxyadenosine
  modified_base (23)..(23): 2'-deoxy-2'-fluorouridine
  modified_base (24)..(24): 2'-methoxyuridine
  modified_base (25)..(25): 2'-deoxy-2'-fluorouridine
auauaagccagacuuuguuggauuu

SEQ ID NO: 6 - RNA, 27 nt, Artificial Sequence
  HPRT1_ssRNA6
  modified_base (1)..(1): 2'-deoxy-2'-fluoroguanosine
  misc_feature (1)..(2): 5'-phosphorothioated
  modified_base (2)..(2): 2'-methoxyguanosine
  misc_feature (2)..(3): 5'-phosphorothioated
  modified_base (3)..(3): 2'-deoxy-2'-fluoroadenosine
  modified_base (4)..(4): 2'-methoxyuridine
  modified_base (5)..(5): 2'-deoxy-2'-fluoroadenosine
  modified_base (6)..(6): 2'-methoxyuridine
  modified_base (7)..(7): 2'-deoxy-2'-fluoroadenosine
  modified_base (8)..(8): 2'-methoxyadenosine
  modified_base (9)..(9): 2'-deoxy-2'-fluoroguanosine
  modified_base (10)..(10): 2'-methoxycytidine
  modified_base (11)..(11): 2'-deoxy-2'-fluorocytidine
  modified_base (12)..(12): 2'-methoxyadenosine
  modified_base (13)..(13): 2'-deoxy-2'-fluoroguanosine
  modified_base (14)..(14): 2'-methoxyadenosine
  modified_base (15)..(15): 2'-deoxy-2'-fluorocytidine
  modified_base (16)..(16): 2'-methoxyuridine
  modified_base (17)..(17): 2'-deoxy-2'-fluorouridine
  modified_base (18)..(18): 2'-methoxyuridine
  modified_base (19)..(19): 2'-deoxy-2'-fluoroguanosine
  modified_base (20)..(20): 2'-methoxyuridine
  modified_base (21)..(21): 2'-deoxy-2'-fluorouridine
  modified_base (22)..(22): 2'-methoxyguanosine
  modified_base (23)..(23): 2'-deoxy-2'-fluoroguanosine
  modified_base (24)..(24): 2'-methoxyadenosine
  modified_base (25)..(25): 2'-deoxy-2'-fluorouridine
  modified_base (26)..(26): 2'-methoxyuridine
  modified_base (27)..(27): 2'-deoxy-2'-fluorouridine
ggauauaagccagacuuuguuggauuu

SEQ ID NO: 7 - RNA, 27 nt, Artificial Sequence
  HPRT1_ssRNA7
  modified_base (1)..(1): 2'-deoxy-2'-fluoroadenosine
  misc_feature (1)..(2): 5'-phosphorothioated
  modified_base (2)..(2): 2'-methoxyuridine
  misc_feature (2)..(3): 5'-phosphorothioated
  modified_base (3)..(3): 2'-deoxy-2'-fluorocytidine
  modified_base (4)..(4): 2'-methoxycytidine
  modified_base (5)..(5): 2'-deoxy-2'-fluoroadenosine
  modified_base (6)..(6): 2'-methoxyuridine
  modified_base (7)..(7): 2'-deoxy-2'-fluorouridine
  modified_base (8)..(8): 2'-methoxycytidine
  modified_base (9)..(9): 2'-deoxy-2'-fluorocytidine
  modified_base (10)..(10): 2'-methoxyuridine
  modified_base (11)..(11): 2'-deoxy-2'-fluoroadenosine
  modified_base (12)..(12): 2'-methoxyuridine
  modified_base (13)..(13): 2'-deoxy-2'-fluoroguanosine
  modified_base (14)..(14): 2'-methoxyadenosine
  modified_base (15)..(15): 2'-deoxy-2'-fluorocytidine
  modified_base (16)..(16): 2'-methoxyuridine
  modified_base (17)..(17): 2'-deoxy-2'-fluoroguanosine
  modified_base (18)..(18): 2'-methoxyuridine
  modified_base (19)..(19): 2'-deoxy-2'-fluoroadenosine
  modified_base (20)..(20): 2'-methoxyguanosine
  modified_base (21)..(21): 2'-deoxy-2'-fluoroadenosine
  modified_base (22)..(22): 2'-methoxyuridine
  modified_base (23)..(23): 2'-deoxy-2'-fluorouridine
  modified_base (24)..(24): 2'-methoxyuridine
  modified_base (25)..(25): 2'-deoxy-2'-fluorouridine
  misc_feature (25)..(26): 5'-phosphorothioated
  modified_base (26)..(26): 2'-methoxyadenosine
  misc_feature (26)..(27): 5'-phosphorothioated
  modified_base (27)..(27): 2'-deoxy-2'-fluorouridine
auccauuccuaugacuguagauuuuau

SEQ ID NO: 8 - RNA, 21 nt, Artificial Sequence
  HPRT1_asRNA1
  modified_base (1)..(1): 2'-methoxyadenosine
  misc_feature (1)..(2): 5'-phosphorothioated
  modified_base (2)..(2): 2'-deoxy-2'-fluoroadenosine
  misc_feature (2)..(3): 5'-phosphorothioated
  modified_base (3)..(3): 2'-methoxyadenosine
  modified_base (4)..(4): 2'-deoxy-2'-fluorouridine
  modified_base (5)..(5): 2'-methoxycytidine
  modified_base (6)..(6): 2'-deoxy-2'-fluorocytidine
  modified_base (7)..(7): 2'-methoxyadenosine
  modified_base (8)..(8): 2'-deoxy-2'-fluoroadenosine
  modified_base (9)..(9): 2'-methoxycytidine
  modified_base (10)..(10): 2'-deoxy-2'-fluoroadenosine
  modified_base (11)..(11): 2'-methoxyadenosine
  modified_base (12)..(12): 2'-deoxy-2'-fluoroadenosine
  modified_base (13)..(13): 2'-methoxyguanosine
  modified_base (14)..(14): 2'-deoxy-2'-fluorouridine
  modified_base (15)..(15): 2'-methoxycytidine
  modified_base (16)..(16): 2'-deoxy-2'-fluorouridine
  modified_base (17)..(17): 2'-methoxyguanosine
  modified_base (18)..(18): 2'-deoxy-2'-fluoroguanosine
  modified_base (19)..(19): 2'-methoxycytidine
  misc_feature (19)..(20): 5'-phosphorothioated
  modified_base (20)..(20): 2'-deoxy-2'-fluorouridine
  misc_feature (20)..(21): 5'-phosphorothioated
  modified_base (21)..(21): 2'-methoxyuridine
aaauccaacaaagucuggcuu

SEQ ID NO: 9 - RNA, 22 nt, Artificial Sequence
  HPRT1_asRNA2
  modified_base (1)..(1): 2'-methoxyadenosine
  misc_feature (1)..(2): 5'-phosphorothioated
  modified_base (2)..(2): 2'-deoxy-2'-fluoroadenosine
  misc_feature (2)..(3): 5'-phosphorothioated
  modified_base (3)..(3): 2'-methoxyadenosine
  modified_base (4)..(4): 2'-deoxy-2'-fluorouridine
  modified_base (5)..(5): 2'-methoxycytidine
  modified_base (6)..(6): 2'-deoxy-2'-fluorocytidine
  modified_base (7)..(7): 2'-methoxyadenosine
  modified_base (8)..(8): 2'-deoxy-2'-fluoroadenosine
  modified_base (9)..(9): 2'-methoxycytidine
  modified_base (10)..(10): 2'-deoxy-2'-fluoroadenosine
  modified_base (11)..(11): 2'-methoxyadenosine
  modified_base (12)..(12): 2'-deoxy-2'-fluoroadenosine
  modified_base (13)..(13): 2'-methoxyguanosine
  modified_base (14)..(14): 2'-deoxy-2'-fluorouridine
  modified_base (15)..(15): 2'-methoxycytidine
  modified_base (16)..(16): 2'-deoxy-2'-fluorouridine
  modified_base (17)..(17): 2'-methoxyguanosine
  modified_base (18)..(18): 2'-deoxy-2'-fluoroguanosine
  modified_base (19)..(19): 2'-methoxycytidine
  modified_base (20)..(20): 2'-deoxy-2'-fluorouridine
  modified_base (21)..(21): 2'-methoxyuridine
  misc_feature (21)..(22): 5'-phosphorothioated
  modified_base (22)..(22): 2'-deoxy-2'-fluoroadenosine
aaauccaacaaagucuggcuua

SEQ ID NO: 10 - RNA, 21 nt, Artificial Sequence
  HPRT1_asRNA3
  modified_base (1)..(1): 2'-methoxyadenosine
  modified_base (2)..(2): 2'-deoxy-2'-fluorouridine
  modified_base (3)..(3): 2'-methoxyadenosine
  modified_base (4)..(4): 2'-deoxy-2'-fluoroadenosine
  modified_base (5)..(5): 2'-methoxyadenosine
  modified_base (6)..(6): 2'-deoxy-2'-fluoroadenosine
  modified_base (7)..(7): 2'-methoxyuridine
  modified_base (8)..(8): 2'-deoxy-2'-fluorocytidine
  modified_base (9)..(9): 2'-methoxyuridine
  modified_base (10)..(10): 2'-deoxy-2'-fluoroadenosine
  modified_base (11)..(11): 2'-methoxycytidine
  modified_base (12)..(12): 2'-deoxy-2'-fluoroadenosine
  modified_base (13)..(13): 2'-methoxyguanosine
  modified_base (14)..(14): 2'-deoxy-2'-fluorouridine
  modified_base (15)..(15): 2'-methoxycytidine
  modified_base (16)..(16): 2'-deoxy-2'-fluoroadenosine
  modified_base (17)..(17): 2'-methoxyuridine
  modified_base (18)..(18): 2'-deoxy-2'-fluoroadenosine
  modified_base (19)..(19): 2'-methoxyguanosine
  misc_feature (19)..(20): 5'-phosphorothioated
  modified_base (20)..(20): 2'-deoxy-2'-fluoroguanosine
  misc_feature (20)..(21): 5'-phosphorothioated
  modified_base (21)..(21): 2'-methoxyadenosine
auaaaaucuacagucauagga

SEQ ID NO: 11 - RNA, 23 nt, Artificial Sequence
  HPRT1_asRNA4
  modified_base (1)..(1): 2'-methoxyadenosine
  modified_base (2)..(2): 2'-deoxy-2'-fluorouridine
  modified_base (3)..(3): 2'-methoxyadenosine
  modified_base (4)..(4): 2'-deoxy-2'-fluoroadenosine
  modified_base (5)..(5): 2'-methoxyadenosine
  modified_base (6)..(6): 2'-deoxy-2'-fluoroadenosine
  modified_base (7)..(7): 2'-methoxyuridine
  modified_base (8)..(8): 2'-deoxy-2'-fluorocytidine
  modified_base (9)..(9): 2'-methoxyuridine
  modified_base (10)..(10): 2'-deoxy-2'-fluoroadenosine
  modified_base (11)..(11): 2'-methoxycytidine
  modified_base (12)..(12): 2'-deoxy-2'-fluoroadenosine
  modified_base (13)..(13): 2'-methoxyguanosine
  modified_base (14)..(14): 2'-deoxy-2'-fluorouridine
  modified_base (15)..(15): 2'-methoxycytidine
  modified_base (16)..(16): 2'-deoxy-2'-fluoroadenosine
  modified_base (17)..(17): 2'-methoxyuridine
  modified_base (18)..(18): 2'-deoxy-2'-fluoroadenosine
  modified_base (19)..(19): 2'-methoxyguanosine
  modified_base (20)..(20): 2'-deoxy-2'-fluoroguanosine
  modified_base (21)..(21): 2'-methoxyadenosine
  misc_feature (21)..(22): 5'-phosphorothioated
  modified_base (22)..(22): 2'-deoxy-2'-fluoroadenosine
  misc_feature (22)..(23): 5'-phosphorothioated
  modified_base (23)..(23): 2'-methoxyuridine
auaaaaucuacagucauaggaau

SEQ ID NO: 12 - RNA, 21 nt, Artificial Sequence
  HPRT1_asRNA5
  modified_base (1)..(1): 2'-methoxyadenosine
  misc_feature (1)..(2): 5'-phosphorothioated
  modified_base (2)..(2): 2'-deoxy-2'-fluorouridine
  misc_feature (2)..(3): 5'-phosphorothioated
  modified_base (3)..(3): 2'-methoxyadenosine
  modified_base (4)..(4): 2'-deoxy-2'-fluoroadenosine
  modified_base (5)..(5): 2'-methoxyadenosine
  modified_base (6)..(6): 2'-deoxy-2'-fluoroadenosine
  modified_base (7)..(7): 2'-methoxyuridine
  modified_base (8)..(8): 2'-deoxy-2'-fluorocytidine
  modified_base (9)..(9): 2'-methoxyuridine
  modified_base (10)..(10): 2'-deoxy-2'-fluoroadenosine
  modified_base (11)..(11): 2'-methoxycytidine
  modified_base (12)..(12): 2'-deoxy-2'-fluoroadenosine
  modified_base (13)..(13): 2'-methoxyguanosine
  modified_base (14)..(14): 2'-deoxy-2'-fluorouridine
  modified_base (15)..(15): 2'-methoxycytidine
  modified_base (16)..(16): 2'-deoxy-2'-fluoroadenosine
  modified_base (17)..(17): 2'-methoxyuridine
  modified_base (18)..(18): 2'-deoxy-2'-fluoroadenosine
  modified_base (19)..(19): 2'-methoxyguanosine
  misc_feature (19)..(20): 5'-phosphorothioated
  modified_base (20)..(20): 2'-deoxy-2'-fluoroguanosine
  misc_feature (20)..(21): 5'-phosphorothioated
  modified_base (21)..(21): 2'-methoxyadenosine
auaaaaucuacagucauagga

SEQ ID NO: 13 - RNA, 25 nt, Artificial Sequence
  HPRT1_csRNA1
  modified_base (1)..(1): 2'-deoxy-2'-fluoroadenosine
  misc_feature (1)..(2): 5'-phosphorothioated
  modified_base (2)..(2): 2'-methoxyuridine
  misc_feature (2)..(3): 5'-phosphorothioated
  modified_base (3)..(3): 2'-deoxy-2'-fluoroadenosine
  modified_base (4)..(4): 2'-methoxyuridine
  modified_base (5)..(5): 2'-deoxy-2'-fluoroadenosine
  modified_base (6)..(6): 2'-methoxyadenosine
  modified_base (7)..(7): 2'-deoxy-2'-fluoroguanosine
  modified_base (8)..(8): 2'-methoxycytidine
  modified_base (9)..(9): 2'-deoxy-2'-fluorocytidine
  modified_base (10)..(10): 2'-methoxyadenosine
  modified_base (11)..(11): 2'-deoxy-2'-fluoroguanosine
  modified_base (12)..(12): 2'-methoxyadenosine
  modified_base (13)..(13): 2'-deoxy-2'-fluorocytidine
  modified_base (14)..(14): 2'-methoxyuridine
  modified_base (15)..(15): 2'-deoxy-2'-fluorouridine
  modified_base (16)..(16): 2'-methoxyuridine
  modified_base (17)..(17): 2'-deoxy-2'-fluoroguanosine
  modified_base (18)..(18): 2'-methoxyuridine
  modified_base (19)..(19): 2'-deoxy-2'-fluorouridine
  modified_base (20)..(20): 2'-methoxyguanosine
  modified_base (21)..(21): 2'-deoxy-2'-fluoroguanosine
  modified_base (22)..(22): 2'-methoxyadenosine
  modified_base (23)..(23): 2'-deoxy-2'-fluorouridine
  modified_base (24)..(24): 2'-methoxyuridine
  modified_base (25)..(25): 2'-deoxy-2'-fluorouridine
auauaagccagacuuuguuggauuu

SEQ ID NO: 14 - RNA, 27 nt, Artificial Sequence
  HPRT1_csRNA2
  modified_base (1)..(1): 2'-deoxy-2'-fluoroguanosine
  misc_feature (1)..(2): 5'-phosphorothioated
  modified_base (2)..(2): 2'-methoxyguanosine
  misc_feature (2)..(3): 5'-phosphorothioated
  modified_base (3)..(3): 2'-deoxy-2'-fluoroadenosine
  modified_base (4)..(4): 2'-methoxyuridine
  modified_base (5)..(5): 2'-deoxy-2'-fluoroadenosine
  modified_base (6)..(6): 2'-methoxyuridine
  modified_base (7)..(7): 2'-deoxy-2'-fluoroadenosine
  modified_base (8)..(8): 2'-methoxyadenosine
  modified_base (9)..(9): 2'-deoxy-2'-fluoroguanosine
  modified_base (10)..(10): 2'-methoxycytidine
  modified_base (11)..(11): 2'-deoxy-2'-fluorocytidine
  modified_base (12)..(12): 2'-methoxyadenosine
  modified_base (13)..(13): 2'-deoxy-2'-fluoroguanosine
  modified_base (14)..(14): 2'-methoxyadenosine
  modified_base (15)..(15): 2'-deoxy-2'-fluorocytidine
  modified_base (16)..(16): 2'-methoxyuridine
  modified_base (17)..(17): 2'-deoxy-2'-fluorouridine
  modified_base (18)..(18): 2'-methoxyuridine
  modified_base (19)..(19): 2'-deoxy-2'-fluoroguanosine
  modified_base (20)..(20): 2'-methoxyuridine
  modified_base (21)..(21): 2'-deoxy-2'-fluorouridine
  modified_base (22)..(22): 2'-methoxyguanosine
  modified_base (23)..(23): 2'-deoxy-2'-fluoroguanosine
  modified_base (24)..(24): 2'-methoxyadenosine
  modified_base (25)..(25): 2'-deoxy-2'-fluorouridine
  modified_base (26)..(26): 2'-methoxyuridine
  modified_base (27)..(27): 2'-deoxy-2'-fluorouridine
ggauauaagccagacuuuguuggauuu

SEQ ID NO: 15 - RNA, 25 nt, Artificial Sequence
  HPRT1_csRNA3
  modified_base (1)..(1): 2'-deoxy-2'-fluorocytidine
  modified_base (2)..(2): 2'-methoxycytidine
  modified_base (3)..(3): 2'-deoxy-2'-fluoroadenosine
  modified_base (4)..(4): 2'-methoxyuridine
  modified_base (5)..(5): 2'-deoxy-2'-fluorouridine
  modified_base (6)..(6): 2'-methoxycytidine
  modified_base (7)..(7): 2'-deoxy-2'-fluorocytidine
  modified_base (8)..(8): 2'-methoxyuridine
  modified_base (9)..(9): 2'-deoxy-2'-fluoroadenosine
  modified_base (10)..(10): 2'-methoxyuridine
  modified_base (11)..(11): 2'-deoxy-2'-fluoroguanosine
  modified_base (12)..(12): 2'-methoxyadenosine
  modified_base (13)..(13): 2'-deoxy-2'-fluorocytidine
  modified_base (14)..(14): 2'-methoxyuridine
  modified_base (15)..(15): 2'-deoxy-2'-fluoroguanosine
  modified_base (16)..(16): 2'-methoxyuridine
  modified_base (17)..(17): 2'-deoxy-2'-fluoroadenosine
  modified_base (18)..(18): 2'-methoxyguanosine
  modified_base (19)..(19): 2'-deoxy-2'-fluoroadenosine
  modified_base (20)..(20): 2'-methoxyuridine
  modified_base (21)..(21): 2'-deoxy-2'-fluorouridine
  modified_base (22)..(22): 2'-methoxyuridine
  modified_base (23)..(23): 2'-deoxy-2'-fluorouridine
  modified_base (24)..(24): 2'-methoxyadenosine
  modified_base (25)..(25): 2'-deoxy-2'-fluorouridine
ccauuccuaugacuguagauuuuau

SEQ ID NO: 16 - RNA, 27 nt, Artificial Sequence
  HPRT1_csRNA4
  modified_base (1)..(1): 2'-deoxy-2'-fluoroadenosine
  modified_base (2)..(2): 2'-methoxyuridine
  modified_base (3)..(3): 2'-deoxy-2'-fluorocytidine
  modified_base (4)..(4): 2'-methoxycytidine
  modified_base (5)..(5): 2'-deoxy-2'-fluoroadenosine
  modified_base (6)..(6): 2'-methoxyuridine
  modified_base (7)..(7): 2'-deoxy-2'-fluorouridine
  modified_base (8)..(8): 2'-methoxycytidine
  modified_base (9)..(9): 2'-deoxy-2'-fluorocytidine
  modified_base (10)..(10): 2'-methoxyuridine
  modified_base (11)..(11): 2'-deoxy-2'-fluoroadenosine
  modified_base (12)..(12): 2'-methoxyuridine
  modified_base (13)..(13): 2'-deoxy-2'-fluoroguanosine
  modified_base (14)..(14): 2'-methoxyadenosine
  modified_base (15)..(15): 2'-deoxy-2'-fluorocytidine
  modified_base (16)..(16): 2'-methoxyuridine
  modified_base (17)..(17): 2'-deoxy-2'-fluoroguanosine
  modified_base (18)..(18): 2'-methoxyuridine
  modified_base (19)..(19): 2'-deoxy-2'-fluoroadenosine
  modified_base (20)..(20): 2'-methoxyguanosine
  modified_base (21)..(21): 2'-deoxy-2'-fluoroadenosine
  modified_base (22)..(22): 2'-methoxyuridine
  modified_base (23)..(23): 2'-deoxy-2'-fluorouridine
  modified_base (24)..(24): 2'-methoxyuridine
  modified_base (25)..(25): 2'-deoxy-2'-fluorouridine
  modified_base (26)..(26): 2'-methoxyadenosine
  modified_base (27)..(27): 2'-deoxy-2'-fluorouridine
auccauuccuaugacuguagauuuuau

SEQ ID NO: 17 - RNA, 27 nt, Artificial Sequence
  HPRT1_csRNA5
  modified_base (1)..(1): 2'-deoxy-2'-fluoroadenosine
  misc_feature (1)..(2): 5'-phosphorothioated
  modified_base (2)..(2): 2'-methoxyuridine
  misc_feature (2)..(3): 5'-phosphorothioated
  modified_base (3)..(3): 2'-deoxy-2'-fluorocytidine
  modified_base (4)..(4): 2'-methoxycytidine
  modified_base (5)..(5): 2'-deoxy-2'-fluoroadenosine
  modified_base (6)..(6): 2'-methoxyuridine
  modified_base (7)..(7): 2'-deoxy-2'-fluorouridine
  modified_base (8)..(8): 2'-methoxycytidine
  modified_base (9)..(9): 2'-deoxy-2'-fluorocytidine
  modified_base (10)..(10): 2'-methoxyuridine
  modified_base (11)..(11): 2'-deoxy-2'-fluoroadenosine
  modified_base (12)..(12): 2'-methoxyuridine
  modified_base (13)..(13): 2'-deoxy-2'-fluoroguanosine
  modified_base (14)..(14): 2'-methoxyadenosine
  modified_base (15)..(15): 2'-deoxy-2'-fluorocytidine
  modified_base (16)..(16): 2'-methoxyuridine
  modified_base (17)..(17): 2'-deoxy-2'-fluoroguanosine
  modified_base (18)..(18): 2'-methoxyuridine
  modified_base (19)..(19): 2'-deoxy-2'-fluoroadenosine
  modified_base (20)..(20): 2'-methoxyguanosine
  modified_base (21)..(21): 2'-deoxy-2'-fluoroadenosine
  modified_base (22)..(22): 2'-methoxyuridine
  modified_base (23)..(23): 2'-deoxy-2'-fluorouridine
  modified_base (24)..(24): 2'-methoxyuridine
  modified_base (25)..(25): 2'-deoxy-2'-fluorouridine
  misc_feature (25)..(26): 5'-phosphorothioated
  modified_base (26)..(26): 2'-methoxyadenosine
  misc_feature (26)..(27): 5'-phosphorothioated
  modified_base (27)..(27): 2'-deoxy-2'-fluorouridine
auccauuccuaugacuguagauuuuau

SEQ ID NO: 18 - RNA, 27 nt, Artificial Sequence
  HRT1_csRNA6
  modified_base (1)..(1): 2'-deoxy-2'-fluorouridine
  misc_feature (1)..(2): 5'-phosphorothioated
  modified_base (2)..(2): 2'-methoxyuridine
  misc_feature (2)..(3): 5'-phosphorothioated
  modified_base (3)..(3): 2'-deoxy-2'-fluorouridine
  modified_base (4)..(4): 2'-methoxyuridine
  modified_base (5)..(5): 2'-deoxy-2'-fluoroadenosine
  modified_base (6)..(6): 2'-methoxyuridine
  modified_base (7)..(7): 2'-deoxy-2'-fluorouridine
  modified_base (8)..(8): 2'-methoxycytidine
  modified_base (9)..(9): 2'-deoxy-2'-fluorocytidine
  modified_base (10)..(10): 2'-methoxyuridine
  modified_base (11)..(11): 2'-deoxy-2'-fluoroadenosine
  modified_base (12)..(12): 2'-methoxyuridine
  modified_base (13)..(13): 2'-deoxy-2'-fluoroguanosine
  modified_base (14)..(14): 2'-methoxyadenosine
  modified_base (15)..(15): 2'-deoxy-2'-fluorocytidine
  modified_base (16)..(16): 2'-methoxyuridine
  modified_base (17)..(17): 2'-deoxy-2'-fluoroguanosine
  modified_base (18)..(18): 2'-methoxyuridine
  modified_base (19)..(19): 2'-deoxy-2'-fluoroadenosine
  modified_base (20)..(20): 2'-methoxyguanosine
  modified_base (21)..(21): 2'-deoxy-2'-fluoroadenosine
  modified_base (22)..(22): 2'-methoxyuridine
  modified_base (23)..(23): 2'-deoxy-2'-fluorouridine
  modified_base (24)..(24): 2'-methoxyuridine
  modified_base (25)..(25): 2'-deoxy-2'-fluorouridine
  misc_feature (25)..(26): 5'-phosphorothioated
  modified_base (26)..(26): 2'-methoxyadenosine
  misc_feature (26)..(27): 5'-phosphorothioated
  modified_base (27)..(27): 2'-deoxy-2'-fluorouridine
uuuuauuccuaugacuguagauuuuau

SEQ ID NO: 19 - RNA, 23 nt, Artificial Sequence
  HPRT1_csRNA7
  modified_base (1)..(1): 2'-deoxy-2'-fluoroadenosine
  misc_feature (1)..(2): 5'-phosphorothioated
  modified_base (2)..(2): 2'-methoxyuridine
  misc_feature (2)..(3): 5'-phosphorothioated
  modified_base (3)..(3): 2'-deoxy-2'-fluorouridine
  modified_base (4)..(4): 2'-methoxycytidine
  modified_base (5)..(5): 2'-deoxy-2'-fluorocytidine
  modified_base (6)..(6): 2'-methoxyuridine
  modified_base (7)..(7): 2'-deoxy-2'-fluoroadenosine
  modified_base (8)..(8): 2'-methoxyuridine
  modified_base (9)..(9): 2'-deoxy-2'-fluoroguanosine
  modified_base (10)..(10): 2'-methoxyadenosine
  modified_base (11)..(11): 2'-deoxy-2'-fluorocytidine
  modified_base (12)..(12): 2'-methoxyuridine
  modified_base (13)..(13): 2'-deoxy-2'-fluoroguanosine
  modified_base (14)..(14): 2'-methoxyuridine
  modified_base (15)..(15): 2'-deoxy-2'-fluoroadenosine
  modified_base (16)..(16): 2'-methoxyguanosine
  modified_base (17)..(17): 2'-deoxy-2'-fluoroadenosine
  modified_base (18)..(18): 2'-methoxyuridine
  modified_base (19)..(19): 2'-deoxy-2'-fluorouridine
  modified_base (20)..(20): 2'-methoxyuridine
  modified_base (21)..(21): 2'-deoxy-2'-fluorouridine
  misc_feature (21)..(22): 5'-phosphorothioated
  modified_base (22)..(22): 2'-methoxyadenosine
  misc_feature (22)..(23): 5'-phosphorothioated
  modified_base (23)..(23): 2'-deoxy-2'-fluorouridine
auuccuaugacuguagauuuuau

SEQ ID NO: 20 - RNA, 22 nt, Artificial Sequence
  HPRT1_csRNA8
  modified_base (1)..(1): 2'-methoxyuridine
  misc_feature (1)..(2): 5'-phosphorothioated
  modified_base (2)..(2): 2'-deoxy-2'-fluorouridine
  modified_base (3)..(3): 2'-methoxycytidine
  modified_base (4)..(4): 2'-deoxy-2'-fluorocytidine
  modified_base (5)..(5): 2'-methoxyuridine
  modified_base (6)..(6): 2'-deoxy-2'-fluoroadenosine
  modified_base (7)..(7): 2'-methoxyuridine
  modified_base (8)..(8): 2'-deoxy-2'-fluoroguanosine
  modified_base (9)..(9): 2'-methoxyadenosine
  modified_base (10)..(10): 2'-deoxy-2'-fluorocytidine
  modified_base (11)..(11): 2'-methoxyuridine
  modified_base (12)..(12): 2'-deoxy-2'-fluoroguanosine
  modified_base (13)..(13): 2'-methoxyuridine
  modified_base (14)..(14): 2'-deoxy-2'-fluoroadenosine
  modified_base (15)..(15): 2'-methoxyguanosine
  modified_base (16)..(16): 2'-deoxy-2'-fluoroadenosine
  modified_base (17)..(17): 2'-methoxyuridine
  modified_base (18)..(18): 2'-deoxy-2'-fluorouridine
  modified_base (19)..(19): 2'-methoxyuridine
  modified_base (20)..(20): 2'-deoxy-2'-fluorouridine
  misc_feature (20)..(21): 5'-phosphorothioated
  modified_base (21)..(21): 2'-methoxyadenosine
  misc_feature (21)..(22): 5'-phosphorothioated
  modified_base (22)..(22): 2'-deoxy-2'-fluorouridine
uuccuaugacuguagauuuuau

SEQ ID NO: 21 - RNA, 23 nt, Artificial Sequence
  HPRT1_csRNA9
  modified_base (1)..(1): 2'-deoxy-2'-fluoroadenosine
  misc_feature (1)..(2): 5'-phosphorothioated
  modified_base (2)..(2): 2'-methoxyuridine
  misc_feature (2)..(3): 5'-phosphorothioated
  modified_base (3)..(3): 2'-deoxy-2'-fluorouridine
  modified_base (4)..(4): 2'-methoxycytidine
  modified_base (5)..(5): 2'-deoxy-2'-fluorocytidine
  modified_base (6)..(6): 2'-methoxyuridine
  modified_base (7)..(7): 2'-deoxy-2'-fluoroadenosine
  modified_base (8)..(8): 2'-methoxyuridine
  modified_base (9)..(9): 2'-deoxy-2'-fluoroguanosine
  modified_base (10)..(10): 2'-methoxyadenosine
  modified_base (11)..(11): 2'-deoxy-2'-fluorocytidine
  modified_base (12)..(12): 2'-methoxyuridine
  modified_base (13)..(13): 2'-deoxy-2'-fluoroguanosine
  modified_base (14)..(14): 2'-methoxyuridine
  modified_base (15)..(15): 2'-deoxy-2'-fluoroadenosine
  modified_base (16)..(16): 2'-methoxyguanosine
  modified_base (17)..(17): 2'-deoxy-2'-fluoroadenosine
  modified_base (18)..(18): 2'-methoxyuridine
  modified_base (19)..(19): 2'-deoxy-2'-fluorouridine
  modified_base (20)..(20): 2'-methoxyuridine
  modified_base (21)..(21): 2'-deoxy-2'-fluorouridine
  misc_feature (21)..(22): 5'-phosphorothioated
  modified_base (22)..(22): 2'-methoxyadenosine
  misc_feature (22)..(23): 5'-phosphorothioated
  modified_base (23)..(23): 2'-deoxy-2'-fluorouridine
auuccuaugacuguagauuuuau

SEQ ID NO: 22 - RNA, 27 nt, Artificial Sequence
  HPRT1_csRNA10
  modified_base (1)..(1): 2'-deoxy-2'-fluoroadenosine
  misc_feature (1)..(2): 5'-phosphorothioated
  modified_base (2)..(2): 2'-methoxyuridine
  misc_feature (2)..(3): 5'-phosphorothioated
  modified_base (3)..(3): 2'-deoxy-2'-fluorocytidine
  modified_base (4)..(4): 2'-methoxycytidine
  modified_base (5)..(5): 2'-deoxy-2'-fluoroadenosine
  modified_base (6)..(6): 2'-methoxyuridine
  modified_base (7)..(7): 2'-deoxy-2'-fluorouridine
  modified_base (8)..(8): 2'-methoxycytidine
  modified_base (9)..(9): 2'-deoxy-2'-fluorocytidine
  modified_base (10)..(10): 2'-methoxyuridine
  modified_base (11)..(11): 2'-deoxy-2'-fluoroadenosine
  modified_base (12)..(12): 2'-methoxyuridine
  modified_base (13)..(13): 2'-deoxy-2'-fluoroguanosine
  modified_base (14)..(14): 2'-methoxyadenosine
  modified_base (15)..(15): 2'-deoxy-2'-fluorocytidine
  modified_base (16)..(16): 2'-methoxyuridine
  modified_base (17)..(17): 2'-deoxy-2'-fluoroguanosine
  modified_base (18)..(18): 2'-methoxyuridine
  modified_base (19)..(19): 2'-deoxy-2'-fluoroadenosine
  modified_base (20)..(20): 2'-methoxyguanosine
  modified_base (21)..(21): 2'-deoxy-2'-fluoroadenosine
  modified_base (22)..(22): 2'-methoxyuridine
  modified_base (23)..(23): 2'-deoxy-2'-fluorouridine
  modified_base (24)..(24): 2'-methoxyuridine
  modified_base (25)..(25): 2'-deoxy-2'-fluorouridine
  misc_feature (25)..(26): 5'-phosphorothioated
  modified_base (26)..(26): 2'-methoxyadenosine
  misc_feature (26)..(27): 5'-phosphorothioated
  modified_base (27)..(27): 2'-deoxy-2'-fluorouridine
auccauuccuaugacuguagauuuuau

SEQ ID NO: 23 - RNA, 26 nt, Artificial Sequence
  HPRT1_csRNA11
  modified_base (1)..(1): 2'-methoxyuridine
  misc_feature (1)..(2): 5'-phosphorothioated
  modified_base (2)..(2): 2'-deoxy-2'-fluorocytidine
  modified_base (3)..(3): 2'-methoxycytidine
  modified_base (4)..(4): 2'-deoxy-2'-fluoroadenosine
  modified_base (5)..(5): 2'-methoxyuridine
  modified_base (6)..(6): 2'-deoxy-2'-fluorouridine
  modified_base (7)..(7): 2'-methoxycytidine
  modified_base (8)..(8): 2'-deoxy-2'-fluorocytidine
  modified_base (9)..(9): 2'-methoxyuridine
  modified_base (10)..(10): 2'-deoxy-2'-fluoroadenosine
  modified_base (11)..(11): 2'-methoxyuridine
  modified_base (12)..(12): 2'-deoxy-2'-fluoroguanosine
  modified_base (13)..(13): 2'-methoxyadenosine
  modified_base (14)..(14): 2'-deoxy-2'-fluorocytidine
  modified_base (15)..(15): 2'-methoxyuridine
  modified_base (16)..(16): 2'-deoxy-2'-fluoroguanosine
  modified_base (17)..(17): 2'-methoxyuridine
  modified_base (18)..(18): 2'-deoxy-2'-fluoroadenosine
  modified_base (19)..(19): 2'-methoxyguanosine
  modified_base (20)..(20): 2'-deoxy-2'-fluoroadenosine
  modified_base (21)..(21): 2'-methoxyuridine
  modified_base (22)..(22): 2'-deoxy-2'-fluorouridine
  modified_base (23)..(23): 2'-methoxyuridine
  modified_base (24)..(24): 2'-deoxy-2'-fluorouridine
  misc_feature (24)..(25): 5'-phosphorothioated
  modified_base (25)..(25): 2'-methoxyadenosine
  misc_feature (25)..(26): 5'-phosphorothioated
  modified_base (26)..(26): 2'-deoxy-2'-fluorouridine
uccauuccuaugacuguagauuuuau

SEQ ID NO: 24 - RNA, 26 nt, Artificial Sequence
  HPRT1_csRNA12
  modified_base (1)..(1): 2'-methoxyuridine
  misc_feature (1)..(2): 5'-phosphorothioated
  modified_base (2)..(2): 2'-deoxy-2'-fluorocytidine
  modified_base (3)..(3): 2'-methoxycytidine
  modified_base (4)..(4): 2'-deoxy-2'-fluoroadenosine
  modified_base (5)..(5): 2'-methoxyuridine
  modified_base (6)..(6): 2'-deoxy-2'-fluorouridine
  modified_base (7)..(7): 2'-methoxycytidine
  modified_base (8)..(8): 2'-deoxy-2'-fluorocytidine
  modified_base (9)..(9): 2'-methoxyuridine
  modified_base (10)..(10): 2'-deoxy-2'-fluoroadenosine
  modified_base (11)..(11): 2'-methoxyuridine
  modified_base (12)..(12): 2'-deoxy-2'-fluoroguanosine
  modified_base (13)..(13): 2'-methoxyadenosine
  modified_base (14)..(14): 2'-deoxy-2'-fluorocytidine
  modified_base (15)..(15): 2'-methoxyuridine
  modified_base (16)..(16): 2'-deoxy-2'-fluoroguanosine
  modified_base (17)..(17): 2'-methoxyuridine
  modified_base (18)..(18): 2'-deoxy-2'-fluoroadenosine
  modified_base (19)..(19): 2'-methoxyguanosine
  modified_base (20)..(20): 2'-deoxy-2'-fluoroadenosine
  modified_base (21)..(21): 2'-methoxyuridine
  modified_base (22)..(22): 2'-deoxy-2'-fluorouridine
  modified_base (23)..(23): 2'-methoxyuridine
  modified_base (24)..(24): 2'-deoxy-2'-fluorouridine
  misc_feature (24)..(25): 5'-phosphorothioated
  modified_base (25)..(25): 2'-methoxyadenosine
  misc_feature (25)..(26): 5'-phosphorothioated
  modified_base (26)..(26): 2'-deoxy-2'-fluorouridine
uccauuccuaugacuguagauuuuau

SEQ ID NO: 25 - RNA, 27 nt, Artificial Sequence
  HPRT1_csRNA13
  modified_base (1)..(1): 2'-deoxy-2'-fluoroadenosine
  misc_feature (1)..(2): 5'-phosphorothioated
  modified_base (2)..(2): 2'-methoxyuridine
  misc_feature (2)..(3): 5'-phosphorothioated
  modified_base (3)..(3): 2'-deoxy-2'-fluorocytidine
  modified_base (4)..(4): 2'-methoxycytidine
  modified_base (5)..(5): 2'-deoxy-2'-fluoroadenosine
  modified_base (6)..(6): 2'-methoxyuridine
  modified_base (7)..(7): 2'-deoxy-2'-fluorouridine
  modified_base (8)..(8): 2'-methoxycytidine
  modified_base (9)..(9): 2'-deoxy-2'-fluorocytidine
  modified_base (10)..(10): 2'-methoxyuridine
  modified_base (11)..(11): 2'-deoxy-2'-fluoroadenosine
  modified_base (12)..(12): 2'-methoxyuridine
  modified_base (13)..(13): 2'-deoxy-2'-fluoroguanosine
  modified_base (14)..(14): 2'-methoxyadenosine
  modified_base (15)..(15): 2'-deoxy-2'-fluorocytidine
  modified_base (16)..(16): 2'-methoxyuridine
  modified_base (17)..(17): 2'-deoxy-2'-fluoroguanosine
  modified_base (18)..(18): 2'-methoxyuridine
  modified_base (19)..(19): 2'-deoxy-2'-fluoroadenosine
  modified_base (20)..(20): 2'-methoxyguanosine
  modified_base (21)..(21): 2'-deoxy-2'-fluoroadenosine
  modified_base (22)..(22): 2'-methoxyuridine
  modified_base (23)..(23): 2'-deoxy-2'-fluorouridine
  modified_base (24)..(24): 2'-methoxyuridine
  modified_base (25)..(25): 2'-deoxy-2'-fluorouridine
  misc_feature (25)..(26): 5'-phosphorothioated
  modified_base (26)..(26): 2'-methoxyadenosine
  misc_feature (26)..(27): 5'-phosphorothioated
  modified_base (27)..(27): 2'-deoxy-2'-fluorouridine
auccauuccuaugacuguagauuuuau

SEQ ID NO: 26 - RNA, 27 nt, Artificial Sequence
  HPRT1_csRNA14
  modified_base (1)..(1): 2'-deoxy-2'-fluoroadenosine
  misc_feature (1)..(2): 5'-phosphorothioated
  modified_base (2)..(2): 2'-methoxyuridine
  misc_feature (2)..(3): 5'-phosphorothioated
  modified_base (3)..(3): 2'-deoxy-2'-fluorocytidine
  modified_base (4)..(4): 2'-methoxycytidine
  modified_base (5)..(5): 2'-deoxy-2'-fluoroadenosine
  modified_base (6)..(6): 2'-methoxyuridine
  modified_base (7)..(7): 2'-deoxy-2'-fluorouridine
  modified_base (8)..(8): 2'-methoxycytidine
  modified_base (9)..(9): 2'-deoxy-2'-fluorocytidine
  modified_base (10)..(10): 2'-methoxyuridine
  modified_base (11)..(11): 2'-deoxy-2'-fluoroadenosine
  modified_base (12)..(12): 2'-methoxyuridine
  modified_base (13)..(13): 2'-deoxy-2'-fluoroguanosine
  modified_base (14)..(14): 2'-methoxyadenosine
  modified_base (15)..(15): 2'-deoxy-2'-fluorocytidine
  modified_base (16)..(16): 2'-methoxyuridine
  modified_base (17)..(17): 2'-deoxy-2'-fluoroguanosine
  modified_base (18)..(18): 2'-methoxyuridine
  modified_base (19)..(19): 2'-deoxy-2'-fluoroadenosine
  modified_base (20)..(20): 2'-methoxyguanosine
  modified_base (21)..(21): 2'-deoxy-2'-fluoroadenosine
  modified_base (22)..(22): 2'-methoxyuridine
  modified_base (23)..(23): 2'-deoxy-2'-fluorouridine
  modified_base (24)..(24): 2'-methoxyuridine
  modified_base (25)..(25): 2'-deoxy-2'-fluorouridine
  misc_feature (25)..(26): 5'-phosphorothioated
  modified_base (26)..(26): 2'-methoxyadenosine
  misc_feature (26)..(27): 5'-phosphorothioated
  modified_base (27)..(27): 2'-deoxy-2'-fluorouridine
auccauuccuaugacuguagauuuuau

SEQ ID NO: 27 - RNA, 27 nt, Artificial Sequence
  HPRT1_csRNA15
  modified_base (1)..(1): 2'-deoxy-2'-fluoroadenosine
  misc_feature (1)..(2): 5'-phosphorothioated
  modified_base (2)..(2): 2'-methoxyuridine
  misc_feature (2)..(3): 5'-phosphorothioated
  modified_base (3)..(3): 2'-deoxy-2'-fluorocytidine
  misc_feature (3)..(4): 5'-phosphorothioated
  modified_base (4)..(4): 2'-methoxycytidine
  misc_feature (4)..(5): 5'-phosphorothioated
  modified_base (5)..(5): 2'-deoxy-2'-fluoroadenosine
  misc_feature (5)..(6): 5'-phosphorothioated
  modified_base (6)..(6): 2'-methoxyuridine
  misc_feature (6)..(7): 5'-phosphorothioated
  modified_base (7)..(7): 2'-deoxy-2'-fluorouridine
  misc_feature (7)..(8): 5'-phosphorothioated
  modified_base (8)..(8): 2'-methoxycytidine
  modified_base (9)..(9): 2'-deoxy-2'-fluorocytidine
  modified_base (10)..(10): 2'-methoxyuridine
  modified_base (11)..(11): 2'-deoxy-2'-fluoroadenosine
  modified_base (12)..(12): 2'-methoxyuridine
  modified_base (13)..(13): 2'-deoxy-2'-fluoroguanosine
  modified_base (14)..(14): 2'-methoxyadenosine
  modified_base (15)..(15): 2'-deoxy-2'-fluorocytidine
  modified_base (16)..(16): 2'-methoxyuridine
  modified_base (17)..(17): 2'-deoxy-2'-fluoroguanosine
  modified_base (18)..(18): 2'-methoxyuridine
  modified_base (19)..(19): 2'-deoxy-2'-fluoroadenosine
  misc_feature (19)..(20): 5'-phosphorothioated
  modified_base (20)..(20): 2'-methoxyguanosine
  misc_feature (20)..(21): 5'-phosphorothioated
  modified_base (21)..(21): 2'-deoxy-2'-fluoroadenosine
  misc_feature (21)..(22): 5'-phosphorothioated
  modified_base (22)..(22): 2'-methoxyuridine
  misc_feature (22)..(23): 5'-phosphorothioated
  modified_base (23)..(23): 2'-deoxy-2'-fluorouridine
  misc_feature (23)..(24): 5'-phosphorothioated
  modified_base (24)..(24): 2'-methoxyuridine
  misc_feature (24)..(25): 5'-phosphorothioated
  modified_base (25)..(25): 2'-deoxy-2'-fluorouridine
  misc_feature (25)..(26): 5'-phosphorothioated
  modified_base (26)..(26): 2'-methoxyadenosine
  misc_feature (26)..(27): 5'-phosphorothioated
  modified_base (27)..(27): 2'-deoxy-2'-fluorouridine
auccauuccuaugacuguagauuuuau

SEQ ID NO: 28 - RNA, 27 nt, Artificial Sequence
  HPRT1_csRNA16
  modified_base (1)..(1): 2'-deoxy-2'-fluorouridine
  misc_feature (1)..(2): 5'-phosphorothioated
  modified_base (2)..(2): 2'-methoxyuridine
  misc_feature (2)..(3): 5'-phosphorothioated
  modified_base (3)..(3): 2'-deoxy-2'-fluorouridine
  misc_feature (3)..(4): 5'-phosphorothioated
  modified_base (4)..(4): 2'-methoxyuridine
  misc_feature (4)..(5): 5'-phosphorothioated
  modified_base (5)..(5): 2'-deoxy-2'-fluoroadenosine
  misc_feature (5)..(6): 5'-phosphorothioated
  modified_base (6)..(6): 2'-methoxyuridine
  misc_feature (6)..(7): 5'-phosphorothioated
  modified_base (7)..(7): 2'-deoxy-2'-fluorouridine
  misc_feature (7)..(8): 5'-phosphorothioated
  modified_base (8)..(8): 2'-methoxycytidine
  misc_feature (8)..(9): 5'-phosphorothioated
  modified_base (9)..(9): 2'-deoxy-2'-fluorocytidine
  modified_base (10)..(10): 2'-methoxyuridine
  modified_base (11)..(11): 2'-deoxy-2'-fluoroadenosine
  modified_base (12)..(12): 2'-methoxyuridine
  modified_base (13)..(13): 2'-deoxy-2'-fluoroguanosine
  modified_base (14)..(14): 2'-methoxyadenosine
  modified_base (15)..(15): 2'-deoxy-2'-fluorocytidine
  modified_base (16)..(16): 2'-methoxyuridine
  modified_base (17)..(17): 2'-deoxy-2'-fluoroguanosine
  modified_base (18)..(18): 2'-methoxyuridine
  modified_base (19)..(19): 2'-deoxy-2'-fluoroadenosine
  modified_base (20)..(20): 2'-methoxyguanosine
  misc_feature (20)..(21): 5'-phosphorothioated
  modified_base (21)..(21): 2'-deoxy-2'-fluoroadenosine
  misc_feature (21)..(22): 5'-phosphorothioated
  modified_base (22)..(22): 2'-methoxyuridine
  misc_feature (22)..(23): 5'-phosphorothioated
  modified_base (23)..(23): 2'-deoxy-2'-fluorouridine
  misc_feature (23)..(24): 5'-phosphorothioated
  modified_base (24)..(24): 2'-methoxyuridine
  misc_feature (24)..(25): 5'-phosphorothioated
  modified_base (25)..(25): 2'-deoxy-2'-fluorouridine
  misc_feature (25)..(26): 5'-phosphorothioated
  modified_base (26)..(26): 2'-methoxyadenosine
  misc_feature (26)..(27): 5'-phosphorothioated
  modified_base (27)..(27): 2'-deoxy-2'-fluorouridine
uuuuauuccuaugacuguagauuuuau

SEQ ID NO: 29 - RNA, 27 nt, Artificial Sequence
  HPRT1_csRNA17
  modified_base (1)..(1): 2'-deoxy-2'-fluoroadenosine
  misc_feature (1)..(2): 5'-phosphorothioated
  modified_base (2)..(2): 2'-methoxyuridine
  misc_feature (2)..(3): 5'-phosphorothioated
  modified_base (3)..(3): 2'-deoxy-2'-fluorocytidine
  misc_feature (3)..(4): 5'-phosphorothioated
  modified_base (4)..(4): 2'-methoxycytidine
  misc_feature (4)..(5): 5'-phosphorothioated
  modified_base (5)..(5): 2'-deoxy-2'-fluoroadenosine
  misc_feature (5)..(6): 5'-phosphorothioated
  modified_base (6)..(6): 2'-methoxyuridine
  misc_feature (6)..(7): 5'-phosphorothioated
  modified_base (7)..(7): 2'-deoxy-2'-fluorouridine
  misc_feature (7)..(8): 5'-phosphorothioated
  modified_base (8)..(8): 2'-methoxycytidine
  misc_feature (8)..(9): 5'-phosphorothioated
  modified_base (9)..(9): 2'-deoxy-2'-fluorocytidine
  modified_base (10)..(10): 2'-methoxyuridine
  modified_base (11)..(11): 2'-deoxy-2'-fluoroadenosine
  modified_base (12)..(12): 2'-methoxyuridine
  modified_base (13)..(13): 2'-deoxy-2'-fluoroguanosine
  modified_base (14)..(14): 2'-methoxyadenosine
  modified_base (15)..(15): 2'-deoxy-2'-fluorocytidine
  modified_base (16)..(16): 2'-methoxyuridine
  modified_base (17)..(17): 2'-deoxy-2'-fluoroguanosine
  modified_base (18)..(18): 2'-methoxyuridine
  modified_base (19)..(19): 2'-deoxy-2'-fluoroadenosine
  modified_base (20)..(20): 2'-methoxyguanosine
  misc_feature (20)..(21): 5'-phosphorothioated
  modified_base (21)..(21): 2'-deoxy-2'-fluoroadenosine
  misc_feature (21)..(22): 5'-phosphorothioated
  modified_base (22)..(22): 2'-methoxyuridine
  misc_feature (22)..(23): 5'-phosphorothioated
  modified_base (23)..(23): 2'-deoxy-2'-fluorouridine
  misc_feature (23)..(24): 5'-phosphorothioated
  modified_base (24)..(24): 2'-methoxyuridine
  misc_feature (24)..(25): 5'-phosphorothioated
  modified_base (25)..(25): 2'-deoxy-2'-fluorouridine
  misc_feature (25)..(26): 5'-phosphorothioated
  modified_base (26)..(26): 2'-methoxyadenosine
  misc_feature (26)..(27): 5'-phosphorothioated
  modified_base (27)..(27): 2'-deoxy-2'-fluorouridine
auccauuccuaugacuguagauuuuau

SEQ ID NO: 30 - RNA, 27 nt, Artificial Sequence
  HPRT1_csRNA18
  modified_base (1)..(1): 2'-deoxy-2'-fluoroadenosine
  misc_feature (1)..(2): 5'-phosphorothioated
  modified_base (2)..(2): 2'-methoxyuridine
  misc_feature (2)..(3): 5'-phosphorothioated
  modified_base (3)..(3): 2'-deoxy-2'-fluorocytidine
  misc_feature (3)..(4): 5'-phosphorothioated
  modified_base (4)..(4): 2'-methoxycytidine
  misc_feature (4)..(5): 5'-phosphorothioated
  modified_base (5)..(5): 2'-deoxy-2'-fluoroadenosine
  misc_feature (5)..(6): 5'-phosphorothioated
  modified_base (6)..(6): 2'-methoxyuridine
  misc_feature (6)..(7): 5'-phosphorothioated
  modified_base (7)..(7): 2'-deoxy-2'-fluorouridine
  misc_feature (7)..(8): 5'-phosphorothioated
  modified_base (8)..(8): 2'-methoxycytidine
  misc_feature (8)..(9): 5'-phosphorothioated
  modified_base (9)..(9): 2'-deoxy-2'-fluorocytidine
  modified_base (10)..(10): 2'-methoxyuridine
  modified_base (11)..(11): 2'-deoxy-2'-fluoroadenosine
  modified_base (12)..(12): 2'-methoxyuridine
  modified_base (13)..(13): 2'-deoxy-2'-fluoroguanosine
  modified_base (14)..(14): 2'-methoxyadenosine
  modified_base (15)..(15): 2'-deoxy-2'-fluorocytidine
  modified_base (16)..(16): 2'-methoxyuridine
  modified_base (17)..(17): 2'-deoxy-2'-fluoroguanosine
  modified_base (18)..(18): 2'-methoxyuridine
  modified_base (19)..(19): 2'-deoxy-2'-fluoroadenosine
  modified_base (20)..(20): 2'-methoxyguanosine
  misc_feature (20)..(21): 5'-phosphorothioated
  modified_base (21)..(21): 2'-deoxy-2'-fluoroadenosine
  misc_feature (21)..(22): 5'-phosphorothioated
  modified_base (22)..(22): 2'-methoxyuridine
  misc_feature (22)..(23): 5'-phosphorothioated
  modified_base (23)..(23): 2'-deoxy-2'-fluorouridine
  misc_feature (23)..(24): 5'-phosphorothioated
  modified_base (24)..(24): 2'-methoxyuridine
  misc_feature (24)..(25): 5'-phosphorothioated
  modified_base (25)..(25): 2'-deoxy-2'-fluorouridine
  misc_feature (25)..(26): 5'-phosphorothioated
  modified_base (26)..(26): 2'-methoxyadenosine
  misc_feature (26)..(27): 5'-phosphorothioated
  modified_base (27)..(27): 2'-deoxy-2'-fluorouridine
auccauuccuaugacuguagauuuuau

SEQ ID NO: 31 - RNA, 25 nt, Artificial Sequence
  HPRT1_csRNA19
  modified_base (1)..(1): 2'-deoxy-2'-fluorouridine
  modified_base (2)..(2): 2'-methoxyuridine
  modified_base (3)..(3): 2'-deoxy-2'-fluoroadenosine
  modified_base (4)..(4): 2'-methoxyuridine
  modified_base (5)..(5): 2'-deoxy-2'-fluorouridine
  modified_base (6)..(6): 2'-methoxycytidine
  modified_base (7)..(7): 2'-deoxy-2'-fluorocytidine
  modified_base (8)..(8): 2'-methoxyuridine
  modified_base (9)..(9): 2'-deoxy-2'-fluoroadenosine
  modified_base (10)..(10): 2'-methoxyuridine
  modified_base (11)..(11): 2'-deoxy-2'-fluoroguanosine
  modified_base (12)..(12): 2'-methoxyadenosine
  modified_base (13)..(13): 2'-deoxy-2'-fluorocytidine
  modified_base (14)..(14): 2'-methoxyuridine
  modified_base (15)..(15): 2'-deoxy-2'-fluoroguanosine
  modified_base (16)..(16): 2'-methoxyuridine
  modified_base (17)..(17): 2'-deoxy-2'-fluoroadenosine
  modified_base (18)..(18): 2'-methoxyguanosine
  modified_base (19)..(19): 2'-deoxy-2'-fluoroadenosine
  modified_base (20)..(20): 2'-methoxyuridine
  modified_base (21)..(21): 2'-deoxy-2'-fluorouridine
  modified_base (22)..(22): 2'-methoxyuridine
  modified_base (23)..(23): 2'-deoxy-2'-fluorouridine
  misc_feature (23)..(24): 5'-phosphorothioated
  modified_base (24)..(24): 2'-methoxyadenosine
  misc_feature (24)..(25): 5'-phosphorothioated
  modified_base (25)..(25): 2'-deoxy-2'-fluorouridine
uuauuccuaugacuguagauuuuau

SEQ ID NO: 32 - RNA, 23 nt, Artificial Sequence
  HPRT1_csRNA20
  modified_base (1)..(1): 2'-deoxy-2'-fluoroadenosine
  misc_feature (1)..(2): 5'-phosphorothioated
  modified_base (2)..(2): 2'-methoxyuridine
  misc_feature (2)..(3): 5'-phosphorothioated
  modified_base (3)..(3): 2'-deoxy-2'-fluorouridine
  misc_feature (3)..(4): 5'-phosphorothioated
  modified_base (4)..(4): 2'-methoxycytidine
  misc_feature (4)..(5): 5'-phosphorothioated
  modified_base (5)..(5): 2'-deoxy-2'-fluorocytidine
  modified_base (6)..(6): 2'-methoxyuridine
  modified_base (7)..(7): 2'-deoxy-2'-fluoroadenosine
  modified_base (8)..(8): 2'-methoxyuridine
  modified_base (9)..(9): 2'-deoxy-2'-fluoroguanosine
  modified_base (10)..(10): 2'-methoxyadenosine
  modified_base (11)..(11): 2'-deoxy-2'-fluorocytidine
  modified_base (12)..(12): 2'-methoxyuridine
  modified_base (13)..(13): 2'-deoxy-2'-fluoroguanosine
  modified_base (14)..(14): 2'-methoxyuridine
  modified_base (15)..(15): 2'-deoxy-2'-fluoroadenosine
  modified_base (16)..(16): 2'-methoxyguanosine
  misc_feature (16)..(17): 5'-phosphorothioated
  modified_base (17)..(17): 2'-deoxy-2'-fluoroadenosine
  misc_feature (17)..(18): 5'-phosphorothioated
  modified_base (18)..(18): 2'-methoxyuridine
  misc_feature (18)..(19): 5'-phosphorothioated
  modified_base (19)..(19): 2'-deoxy-2'-fluorouridine
  misc_feature (19)..(20): 5'-phosphorothioated
  modified_base (20)..(20): 2'-methoxyuridine
  misc_feature (20)..(21): 5'-phosphorothioated
  modified_base (21)..(21): 2'-deoxy-2'-fluorouridine
  misc_feature (21)..(22): 5'-phosphorothioated
  modified_base (22)..(22): 2'-methoxyadenosine
  misc_feature (22)..(23): 5'-phosphorothioated
  modified_base (23)..(23): 2'-deoxy-2'-fluorouridine
auuccuaugacuguagauuuuau

SEQ ID NO: 33 - RNA, 27 nt, Artificial Sequence
  HPRT1_csRNA21
  modified_base (1)..(1): 2'-deoxy-2'-fluoroadenosine
  misc_feature (1)..(2): 5'-phosphorothioated
  modified_base (2)..(2): 2'-methoxyuridine
  misc_feature (2)..(3): 5'-phosphorothioated
  modified_base (3)..(3): 2'-deoxy-2'-fluorocytidine
  modified_base (4)..(4): 2'-methoxycytidine
  modified_base (5)..(5): 2'-deoxy-2'-fluoroadenosine
  modified_base (6)..(6): 2'-methoxyuridine
  modified_base (7)..(7): 2'-deoxy-2'-fluorouridine
  modified_base (8)..(8): 2'-methoxycytidine
  modified_base (9)..(9): 2'-deoxy-2'-fluorocytidine
  modified_base (10)..(10): 2'-methoxyuridine
  modified_base (11)..(11): 2'-deoxy-2'-fluoroadenosine
  modified_base (12)..(12): 2'-methoxyuridine
  modified_base (13)..(13): 2'-deoxy-2'-fluoroguanosine
  modified_base (14)..(14): 2'-methoxyadenosine
  modified_base (15)..(15): 2'-deoxy-2'-fluorocytidine
  modified_base (16)..(16): 2'-methoxyuridine
  modified_base (17)..(17): 2'-deoxy-2'-fluoroguanosine
  modified_base (18)..(18): 2'-methoxyuridine
  modified_base (19)..(19): 2'-deoxy-2'-fluoroadenosine
  modified_base (20)..(20): 2'-methoxyguanosine
  modified_base (21)..(21): 2'-deoxy-2'-fluoroadenosine
  modified_base (22)..(22): 2'-methoxyuridine
  modified_base (23)..(23): 2'-deoxy-2'-fluorouridine
  modified_base (24)..(24): 2'-methoxyuridine
  modified_base (25)..(25): 2'-deoxy-2'-fluorouridine
  misc_feature (25)..(26): 5'-phosphorothioated
  modified_base (26)..(26): 2'-methoxyadenosine
  misc_feature (26)..(27): 5'-phosphorothioated
  modified_base (27)..(27): 2'-deoxy-2'-fluorouridine
auccauuccuaugacuguagauuuuau

SEQ ID NO: 34 - RNA, 27 nt, Artificial Sequence
  HPRT1_csRNA22
  modified_base (1)..(1): 2'-deoxy-2'-fluoroadenosine
  misc_feature (1)..(2): 5'-phosphorothioated
  modified_base (2)..(2): 2'-methoxyuridine
  misc_feature (2)..(3): 5'-phosphorothioated
  modified_base (3)..(3): 2'-deoxy-2'-fluorocytidine
  modified_base (4)..(4): 2'-methoxycytidine
  modified_base (5)..(5): 2'-deoxy-2'-fluoroadenosine
  modified_base (6)..(6): 2'-methoxyuridine
  modified_base (7)..(7): 2'-deoxy-2'-fluorouridine
  modified_base (8)..(8): 2'-methoxycytidine
  modified_base (9)..(9): 2'-deoxy-2'-fluorocytidine
  modified_base (10)..(10): 2'-methoxyuridine
  modified_base (11)..(11): 2'-deoxy-2'-fluoroadenosine
  modified_base (12)..(12): 2'-methoxyuridine
  modified_base (13)..(13): 2'-deoxy-2'-fluoroguanosine
  modified_base (14)..(14): 2'-methoxyadenosine
  modified_base (15)..(15): 2'-deoxy-2'-fluorocytidine
  modified_base (16)..(16): 2'-methoxyuridine
  modified_base (17)..(17): 2'-deoxy-2'-fluoroguanosine
  modified_base (18)..(18): 2'-methoxyuridine
  modified_base (19)..(19): 2'-deoxy-2'-fluoroadenosine
  modified_base (20)..(20): 2'-methoxyguanosine
  modified_base (21)..(21): 2'-deoxy-2'-fluoroadenosine
  modified_base (22)..(22): 2'-methoxyuridine
  modified_base (23)..(23): 2'-deoxy-2'-fluorouridine
  modified_base (24)..(24): 2'-methoxyuridine
  modified_base (25)..(25): 2'-deoxy-2'-fluorouridine
  misc_feature (25)..(26): 5'-phosphorothioated
  modified_base (26)..(26): 2'-methoxyadenosine
  misc_feature (26)..(27): 5'-phosphorothioated
  modified_base (27)..(27): 2'-deoxy-2'-fluorouridine
auccauuccuaugacuguagauuuuau

SEQ ID NO: 35 - RNA, 35 nt, Artificial Sequence
  HPRT1_csRNA23
  modified_base (1)..(1): 2'-methoxyadenosine
  misc_feature (1)..(2): 5'-phosphorothioated
  modified_base (2)..(2): 2'-deoxy-2'-fluoroguanosine
  misc_feature (2)..(3): 5'-phosphorothioated
  modified_base (3)..(3): 2'-methoxyuridine
  modified_base (4)..(4): 2'-deoxy-2'-fluoroguanosine
  modified_base (5)..(5): 2'-deoxy-2'-fluoroadenosine
  modified_base (6)..(6): 2'-methoxyuridine
  modified_base (7)..(7): 2'-deoxy-2'-fluoroadenosine
  modified_base (8)..(8): 2'-methoxyguanosine
  modified_base (9)..(9): 2'-deoxy-2'-fluoroadenosine
  modified_base (10)..(10): 2'-methoxyuridine
  modified_base (11)..(11): 2'-deoxy-2'-fluorocytidine
  modified_base (12)..(12): 2'-methoxycytidine
  modified_base (13)..(13): 2'-deoxy-2'-fluoroadenosine
  modified_base (14)..(14): 2'-methoxyuridine
  modified_base (15)..(15): 2'-deoxy-2'-fluorouridine
  modified_base (16)..(16): 2'-methoxycytidine
  modified_base (17)..(17): 2'-deoxy-2'-fluorocytidine
  modified_base (18)..(18): 2'-methoxyuridine
  modified_base (19)..(19): 2'-deoxy-2'-fluoroadenosine
  modified_base (20)..(20): 2'-methoxyuridine
  modified_base (21)..(21): 2'-deoxy-2'-fluoroguanosine
  modified_base (22)..(22): 2'-methoxyadenosine
  modified_base (23)..(23): 2'-deoxy-2'-fluorocytidine
  modified_base (24)..(24): 2'-methoxyuridine
  modified_base (25)..(25): 2'-deoxy-2'-fluoroguanosine
  modified_base (26)..(26): 2'-methoxyuridine
  modified_base (27)..(27): 2'-deoxy-2'-fluoroadenosine
  modified_base (28)..(28): 2'-methoxyguanosine
  modified_base (29)..(29): 2'-deoxy-2'-fluoroadenosine
  modified_base (30)..(30): 2'-methoxyuridine
  modified_base (31)..(31): 2'-deoxy-2'-fluorouridine
  modified_base (32)..(32): 2'-methoxyuridine
  modified_base (33)..(33): 2'-deoxy-2'-fluorouridine
  misc_feature (33)..(34): 5'-phosphorothioated
  modified_base (34)..(34): 2'-methoxyadenosine
  misc_feature (34)..(35): 5'-phosphorothioated
  modified_base (35)..(35): 2'-deoxy-2'-fluorouridine
agugauagauccauuccuaugacuguagauuuuau

SEQ ID NO: 36 - RNA, 15 nt, Artificial Sequence
  HPRT1_csRNA24
  modified_base (1)..(1): 2'-deoxy-2'-fluoroguanosine
  misc_feature (1)..(2): 5'-phosphorothioated
  modified_base (2)..(2): 2'-methoxyadenosine
  misc_feature (2)..(3): 5'-phosphorothioated
  modified_base (3)..(3): 2'-deoxy-2'-fluorocytidine
  modified_base (4)..(4): 2'-methoxyuridine
  modified_base (5)..(5): 2'-deoxy-2'-fluoroguanosine
  modified_base (6)..(6): 2'-methoxyuridine
  modified_base (7)..(7): 2'-deoxy-2'-fluoroadenosine
  modified_base (8)..(8): 2'-methoxyguanosine
  modified_base (9)..(9): 2'-deoxy-2'-fluoroadenosine
  modified_base (10)..(10): 2'-methoxyuridine
  modified_base (11)..(11): 2'-deoxy-2'-fluorouridine
  modified_base (12)..(12): 2'-methoxyuridine
  modified_base (13)..(13): 2'-deoxy-2'-fluorouridine
  misc_feature (13)..(14): 5'-phosphorothioated
  modified_base (14)..(14): 2'-methoxyadenosine
  misc_feature (14)..(15): 5'-phosphorothioated
  modified_base (15)..(15): 2'-deoxy-2'-fluorouridine
gacuguagauuuuau

SEQ ID NO: 37 - RNA, 27 nt, Artificial Sequence
  HPRT1_csRNA25
  modified_base (1)..(1): 2'-deoxy-2'-fluoroadenosine
  misc_feature (1)..(2): 5'-phosphorothioated
  modified_base (2)..(2): 2'-methoxyuridine
  misc_feature (2)..(3): 5'-phosphorothioated
  modified_base (3)..(3): 2'-deoxy-2'-fluorocytidine
  modified_base (4)..(4): 2'-methoxycytidine
  modified_base (5)..(5): 2'-deoxy-2'-fluoroadenosine
  modified_base (6)..(6): 2'-methoxyuridine
  modified_base (7)..(7): 2'-deoxy-2'-fluorouridine
  modified_base (8)..(8): 2'-methoxycytidine
  modified_base (9)..(9): 2'-deoxy-2'-fluorocytidine
  modified_base (10)..(10): 2'-methoxyuridine
  modified_base (11)..(11): 2'-deoxy-2'-fluoroadenosine
  modified_base (12)..(12): 2'-methoxyuridine
  modified_base (13)..(13): 2'-deoxy-2'-fluoroguanosine
  modified_base (14)..(14): 2'-methoxyadenosine
  modified_base (15)..(15): 2'-deoxy-2'-fluorocytidine
  modified_base (16)..(16): 2'-methoxyuridine
  modified_base (17)..(17): 2'-deoxy-2'-fluoroguanosine
  modified_base (18)..(18): 2'-methoxyuridine
  modified_base (19)..(19): 2'-deoxy-2'-fluoroadenosine
  modified_base (20)..(20): 2'-methoxyguanosine
  modified_base (21)..(21): 2'-deoxy-2'-fluoroadenosine
  modified_base (22)..(22): 2'-methoxyuridine
  modified_base (23)..(23): 2'-deoxy-2'-fluorouridine
  modified_base (24)..(24): 2'-methoxyuridine
  modified_base (25)..(25): 2'-deoxy-2'-fluorouridine
  misc_feature (25)..(26): 5'-phosphorothioated
  modified_base (26)..(26): 2'-methoxyadenosine
  misc_feature (26)..(27): 5'-phosphorothioated
  modified_base (27)..(27): 2'-deoxy-2'-fluorouridine
auccauuccuaugacuguagauuuuau

SEQ ID NO: 38 - RNA, 27 nt, Artificial Sequence
  HPRT1_csRNA26
  modified_base (1)..(1): 2'-deoxy-2'-fluoroadenosine
  misc_feature (1)..(2): 5'-phosphorothioated
  modified_base (2)..(2): 2'-methoxyuridine
  misc_feature (2)..(3): 5'-phosphorothioated
  modified_base (3)..(3): 2'-deoxy-2'-fluorocytidine
  modified_base (4)..(4): 2'-methoxycytidine
  modified_base (5)..(5): 2'-deoxy-2'-fluoroadenosine
  modified_base (6)..(6): 2'-methoxyuridine
  modified_base (7)..(7): 2'-deoxy-2'-fluorouridine
  modified_base (8)..(8): 2'-methoxycytidine
  modified_base (9)..(9): 2'-deoxy-2'-fluorocytidine
  modified_base (10)..(10): 2'-methoxyuridine
  modified_base (11)..(11): 2'-deoxy-2'-fluoroadenosine
  modified_base (12)..(12): 2'-methoxyuridine
  modified_base (13)..(13): 2'-deoxy-2'-fluoroguanosine
  modified_base (14)..(14): 2'-methoxyadenosine
  modified_base (15)..(15): 2'-deoxy-2'-fluorocytidine
  modified_base (16)..(16): 2'-methoxyuridine
  modified_base (17)..(17): 2'-deoxy-2'-fluoroguanosine
  modified_base (18)..(18): 2'-methoxyuridine
  modified_base (19)..(19): 2'-deoxy-2'-fluoroadenosine
  modified_base (20)..(20): 2'-methoxyguanosine
  modified_base (21)..(21): 2'-deoxy-2'-fluoroadenosine
  modified_base (22)..(22): 2'-methoxyuridine
  modified_base (23)..(23): 2'-deoxy-2'-fluorouridine
  modified_base (24)..(24): 2'-methoxyuridine
  modified_base (25)..(25): 2'-deoxy-2'-fluorouridine
  misc_feature (25)..(26): 5'-phosphorothioated
  modified_base (26)..(26): 2'-methoxyadenosine
  misc_feature (26)..(27): 5'-phosphorothioated
  modified_base (27)..(27): 2'-deoxy-2'-fluorouridine
auccauuccuaugacuguagauuuuau

SEQ ID NO: 39 - RNA, 27 nt, Artificial Sequence
  HPRT1_csRNA27
  modified_base (1)..(1): 2'-deoxy-2'-fluoroadenosine
  misc_feature (1)..(2): 5'-phosphorothioated
  modified_base (2)..(2): 2'-methoxyuridine
  misc_feature (2)..(3): 5'-phosphorothioated
  modified_base (3)..(3): 2'-deoxy-2'-fluorocytidine
  modified_base (4)..(4): 2'-methoxycytidine
  modified_base (5)..(5): 2'-deoxy-2'-fluoroadenosine
  modified_base (6)..(6): 2'-methoxyuridine
  modified_base (7)..(7): 2'-deoxy-2'-fluorouridine
  modified_base (8)..(8): 2'-methoxycytidine
  modified_base (9)..(9): 2'-deoxy-2'-fluorocytidine
  modified_base (10)..(10): 2'-methoxyuridine
  modified_base (11)..(11): 2'-deoxy-2'-fluoroadenosine
  modified_base (12)..(12): 2'-methoxyuridine
  modified_base (13)..(13): 2'-deoxy-2'-fluoroguanosine
  modified_base (14)..(14): 2'-methoxyadenosine
  modified_base (15)..(15): 2'-deoxy-2'-fluorocytidine
  modified_base (16)..(16): 2'-methoxyuridine
  modified_base (17)..(17): 2'-deoxy-2'-fluoroguanosine
  modified_base (18)..(18): 2'-methoxyuridine
  modified_base (19)..(19): 2'-deoxy-2'-fluoroadenosine
  modified_base (20)..(20): 2'-methoxyguanosine
  modified_base (21)..(21): 2'-deoxy-2'-fluoroadenosine
  modified_base (22)..(22): 2'-methoxyuridine
  modified_base (23)..(23): 2'-deoxy-2'-fluorouridine
  modified_base (24)..(24): 2'-methoxyuridine
  modified_base (25)..(25): 2'-deoxy-2'-fluorouridine
  misc_feature (25)..(26): 5'-phosphorothioated
  modified_base (26)..(26): 2'-methoxyadenosine
  misc_feature (26)..(27): 5'-phosphorothioated
  modified_base (27)..(27): 2'-deoxy-2'-fluorouridine
auccauuccuaugacuguagauuuuau

SEQ ID NO: 40 - RNA, 27 nt, Artificial Sequence
  HPRT1_csRNA28
  modified_base (1)..(1): 2'-deoxy-2'-fluoroadenosine
  misc_feature (1)..(2): 5'-phosphorothioated
  modified_base (2)..(2): 2'-methoxyuridine
  misc_feature (2)..(3): 5'-phosphorothioated
  modified_base (3)..(3): 2'-deoxy-2'-fluorocytidine
  modified_base (4)..(4): 2'-methoxycytidine
  modified_base (5)..(5): 2'-deoxy-2'-fluoroadenosine
  modified_base (6)..(6): 2'-methoxyuridine
  modified_base (7)..(7): 2'-deoxy-2'-fluorouridine
  modified_base (8)..(8): 2'-methoxycytidine
  modified_base (9)..(9): 2'-deoxy-2'-fluorocytidine
  modified_base (10)..(10): 2'-methoxyuridine
  modified_base (11)..(11): 2'-deoxy-2'-fluoroadenosine
  modified_base (12)..(12): 2'-methoxyuridine
  modified_base (13)..(13): 2'-deoxy-2'-fluoroguanosine
  modified_base (14)..(14): 2'-methoxyadenosine
  modified_base (15)..(15): 2'-deoxy-2'-fluorocytidine
  modified_base (16)..(16): 2'-methoxyuridine
  modified_base (17)..(17): 2'-deoxy-2'-fluoroguanosine
  modified_base (18)..(18): 2'-methoxyuridine
  modified_base (19)..(19): 2'-deoxy-2'-fluoroadenosine
  modified_base (20)..(20): 2'-methoxyguanosine
  modified_base (21)..(21): 2'-deoxy-2'-fluoroadenosine
  modified_base (22)..(22): 2'-methoxyuridine
  modified_base (23)..(23): 2'-deoxy-2'-fluorouridine
  modified_base (24)..(24): 2'-methoxyuridine
  modified_base (25)..(25): 2'-deoxy-2'-fluorouridine
  misc_feature (25)..(26): 5'-phosphorothioated
  modified_base (26)..(26): 2'-methoxyadenosine
  misc_feature (26)..(27): 5'-phosphorothioated
  modified_base (27)..(27): 2'-deoxy-2'-fluorouridine
auccauuccuaugacuguagauuuuau

SEQ ID NO: 41 - RNA, 27 nt, Artificial Sequence
  HPRT1_csRNA29
  modified_base (1)..(1): 2'-deoxy-2'-fluoroadenosine
  misc_feature (1)..(2): 5'-phosphorothioated
  modified_base (2)..(2): 2'-methoxyuridine
  misc_feature (2)..(3): 5'-phosphorothioated
  modified_base (3)..(3): 2'-deoxy-2'-fluorocytidine
  modified_base (4)..(4): 2'-methoxycytidine
  modified_base (5)..(5): 2'-deoxy-2'-fluoroadenosine
  modified_base (6)..(6): 2'-methoxyuridine
  modified_base (7)..(7): 2'-deoxy-2'-fluorouridine
  modified_base (8)..(8): 2'-methoxycytidine
  modified_base (9)..(9): 2'-deoxy-2'-fluorocytidine
  modified_base (10)..(10): 2'-methoxyuridine
  modified_base (11)..(11): 2'-deoxy-2'-fluoroadenosine
  modified_base (12)..(12): 2'-methoxyuridine
  modified_base (13)..(13): 2'-deoxy-2'-fluoroguanosine
  modified_base (14)..(14): 2'-methoxyadenosine
  modified_base (15)..(15): 2'-deoxy-2'-fluorocytidine
  modified_base (16)..(16): 2'-methoxyuridine
  modified_base (17)..(17): 2'-deoxy-2'-fluoroguanosine
  modified_base (18)..(18): 2'-methoxyuridine
  modified_base (19)..(19): 2'-deoxy-2'-fluoroadenosine
  modified_base (20)..(20): 2'-methoxyguanosine
  modified_base (21)..(21): 2'-deoxy-2'-fluoroadenosine
  modified_base (22)..(22): 2'-methoxyuridine
  modified_base (23)..(23): 2'-deoxy-2'-fluorouridine
  modified_base (24)..(24): 2'-methoxyuridine
  modified_base (25)..(25): 2'-deoxy-2'-fluorouridine
  misc_feature (25)..(26): 5'-phosphorothioated
  modified_base (26)..(26): 2'-methoxyadenosine
  misc_feature (26)..(27): 5'-phosphorothioated
  modified_base (27)..(27): 2'-deoxy-2'-fluorouridine
auccauuccuaugacuguagauuuuau

SEQ ID NO: 42 - RNA, 27 nt, Artificial Sequence
  HPRT1_csRNA30
  modified_base (1)..(1): 2'-deoxy-2'-fluoroadenosine
  misc_feature (1)..(2): 5'-phosphorothioated
  modified_base (2)..(2): 2'-methoxyuridine
  misc_feature (2)..(3): 5'-phosphorothioated
  modified_base (3)..(3): 2'-deoxy-2'-fluorocytidine
  modified_base (4)..(4): 2'-methoxycytidine
  modified_base (5)..(5): 2'-deoxy-2'-fluoroadenosine
  modified_base (6)..(6): 2'-methoxyuridine
  modified_base (7)..(7): 2'-deoxy-2'-fluorouridine
  modified_base (8)..(8): 2'-methoxycytidine
  modified_base (9)..(9): 2'-deoxy-2'-fluorocytidine
  modified_base (10)..(10): 2'-methoxyuridine
  modified_base (11)..(11): 2'-deoxy-2'-fluoroadenosine
  modified_base (12)..(12): 2'-methoxyuridine
  modified_base (13)..(13): 2'-deoxy-2'-fluoroguanosine
  modified_base (14)..(14): 2'-methoxyadenosine
  modified_base (15)..(15): 2'-deoxy-2'-fluorocytidine
  modified_base (16)..(16): 2'-methoxyuridine
  modified_base (17)..(17): 2'-deoxy-2'-fluoroguanosine
  modified_base (18)..(18): 2'-methoxyuridine
  modified_base (19)..(19): 2'-deoxy-2'-fluoroadenosine
  modified_base (20)..(20): 2'-methoxyguanosine
  modified_base (21)..(21): 2'-deoxy-2'-fluoroadenosine
  modified_base (22)..(22): 2'-methoxyuridine
  modified_base (23)..(23): 2'-deoxy-2'-fluorouridine
  modified_base (24)..(24): 2'-methoxyuridine
  modified_base (25)..(25): 2'-deoxy-2'-fluorouridine
  misc_feature (25)..(26): 5'-phosphorothioated
  modified_base (26)..(26): 2'-methoxyadenosine
  misc_feature (26)..(27): 5'-phosphorothioated
  modified_base (27)..(27): 2'-deoxy-2'-fluorouridine
auccauuccuaugacuguagauuuuau

SEQ ID NO: 43 - RNA, 27 nt, Artificial Sequence
  HPRT1_csRNA31
  modified_base (1)..(1): 2'-deoxy-2'-fluoroadenosine
  misc_feature (1)..(2): 5'-phosphorothioated
  modified_base (2)..(2): 2'-methoxyuridine
  modified_base (3)..(3): 2'-deoxy-2'-fluorocytidine
  modified_base (4)..(4): 2'-methoxycytidine
  modified_base (5)..(5): 2'-deoxy-2'-fluoroadenosine
  modified_base (6)..(6): 2'-methoxyuridine
  modified_base (7)..(7): 2'-deoxy-2'-fluorouridine
  modified_base (8)..(8): 2'-methoxycytidine
  modified_base (9)..(9): 2'-deoxy-2'-fluorocytidine
  modified_base (10)..(10): 2'-methoxyuridine
  modified_base (11)..(11): 2'-deoxy-2'-fluoroadenosine
  modified_base (12)..(12): 2'-methoxyuridine
  modified_base (13)..(13): 2'-deoxy-2'-fluoroguanosine
  modified_base (14)..(14): 2'-methoxyadenosine
  modified_base (15)..(15): 2'-deoxy-2'-fluorocytidine
  modified_base (16)..(16): 2'-methoxyuridine
  modified_base (17)..(17): 2'-deoxy-2'-fluoroguanosine
  modified_base (18)..(18): 2'-methoxyuridine
  modified_base (19)..(19): 2'-deoxy-2'-fluoroadenosine
  modified_base (20)..(20): 2'-methoxyguanosine
  modified_base (21)..(21): 2'-deoxy-2'-fluoroadenosine
  modified_base (22)..(22): 2'-methoxyuridine
  modified_base (23)..(23): 2'-deoxy-2'-fluorouridine
  modified_base (24)..(24): 2'-methoxyuridine
  modified_base (25)..(25): 2'-deoxy-2'-fluorouridine
  modified_base (26)..(26): 2'-methoxyadenosine
  misc_feature (26)..(27): 5'-phosphorothioated
  modified_base (27)..(27): 2'-deoxy-2'-fluorouridine
auccauuccuaugacuguagauuuuau

SEQ ID NO: 44 - RNA, 27 nt, Artificial Sequence
  HPRT1_csRNA32
  modified_base (1)..(1): 2'-deoxy-2'-fluoroadenosine
  misc_feature (1)..(2): 5'-phosphorothioated
  modified_base (2)..(2): 2'-methoxyuridine
  misc_feature (2)..(3): 5'-phosphorothioated
  modified_base (3)..(3): 2'-deoxy-2'-fluorocytidine
  modified_base (4)..(4): 2'-methoxycytidine
  modified_base (5)..(5): 2'-deoxy-2'-fluoroadenosine
  modified_base (6)..(6): 2'-methoxyuridine
  modified_base (7)..(7): 2'-deoxy-2'-fluorouridine
  modified_base (8)..(8): 2'-methoxycytidine
  modified_base (9)..(9): 2'-deoxy-2'-fluorocytidine
  modified_base (10)..(10): 2'-methoxyuridine
  modified_base (11)..(11): 2'-deoxy-2'-fluoroadenosine
  modified_base (12)..(12): 2'-methoxyuridine
  modified_base (13)..(13): 2'-deoxy-2'-fluoroguanosine
  modified_base (14)..(14): 2'-methoxyadenosine
  modified_base (15)..(15): 2'-deoxy-2'-fluorocytidine
  modified_base (16)..(16): 2'-methoxyuridine
  modified_base (17)..(17): 2'-deoxy-2'-fluoroguanosine
  modified_base (18)..(18): 2'-methoxyuridine
  modified_base (19)..(19): 2'-deoxy-2'-fluoroadenosine
  modified_base (20)..(20): 2'-methoxyguanosine
  modified_base (21)..(21): 2'-deoxy-2'-fluoroadenosine
  modified_base (22)..(22): 2'-methoxyuridine
  modified_base (23)..(23): 2'-deoxy-2'-fluorouridine
  modified_base (24)..(24): 2'-methoxyuridine
  modified_base (25)..(25): 2'-deoxy-2'-fluorouridine
  misc_feature (25)..(26): 5'-phosphorothioated
  modified_base (26)..(26): 2'-methoxyadenosine
  misc_feature (26)..(27): 5'-phosphorothioated
  modified_base (27)..(27): 2'-deoxy-2'-fluorouridine
auccauuccuaugacuguagauuuuau

SEQ ID NO: 45 - RNA, 23 nt, Artificial Sequence
  HPRT1_csRNA33
  modified_base (1)..(1): 2'-deoxy-2'-fluoroadenosine
  misc_feature (1)..(2): 5'-phosphorothioated
  modified_base (2)..(2): 2'-methoxyuridine
  misc_feature (2)..(3): 5'-phosphorothioated
  modified_base (3)..(3): 2'-deoxy-2'-fluorouridine
  modified_base (4)..(4): 2'-methoxycytidine
  modified_base (5)..(5): 2'-deoxy-2'-fluorocytidine
  modified_base (6)..(6): 2'-methoxyuridine
  modified_base (7)..(7): 2'-deoxy-2'-fluoroadenosine
  modified_base (8)..(8): 2'-methoxyuridine
  modified_base (9)..(9): 2'-deoxy-2'-fluoroguanosine
  modified_base (10)..(10): 2'-methoxyadenosine
  modified_base (11)..(11): 2'-deoxy-2'-fluorocytidine
  modified_base (12)..(12): 2'-methoxyuridine
  modified_base (13)..(13): 2'-deoxy-2'-fluoroguanosine
  modified_base (14)..(14): 2'-methoxyuridine
  modified_base (15)..(15): 2'-deoxy-2'-fluoroadenosine
  modified_base (16)..(16): 2'-methoxyguanosine
  modified_base (17)..(17): 2'-deoxy-2'-fluoroadenosine
  modified_base (18)..(18): 2'-methoxyuridine
  modified_base (19)..(19): 2'-deoxy-2'-fluorouridine
  modified_base (20)..(20): 2'-methoxyuridine
  modified_base (21)..(21): 2'-deoxy-2'-fluorouridine
  misc_feature (21)..(22): 5'-phosphorothioated
  modified_base (22)..(22): 2'-methoxyadenosine
  misc_feature (22)..(23): 5'-phosphorothioated
  modified_base (23)..(23): 2'-deoxy-2'-fluorouridine
auuccuaugacuguagauuuuau

SEQ ID NO: 46 - RNA, 23 nt, Artificial Sequence
  HPRT1_csRNA34
  modified_base (1)..(1): 2'-deoxy-2'-fluoroadenosine
  misc_feature (1)..(2): 5'-phosphorothioated
  modified_base (2)..(2): 2'-methoxyuridine
  misc_feature (2)..(3): 5'-phosphorothioated
  modified_base (3)..(3): 2'-deoxy-2'-fluorouridine
  modified_base (4)..(4): 2'-methoxycytidine
  modified_base (5)..(5): 2'-deoxy-2'-fluorocytidine
  modified_base (6)..(6): 2'-methoxyuridine
  modified_base (7)..(7): 2'-deoxy-2'-fluoroadenosine
  modified_base (8)..(8): 2'-methoxyuridine
  modified_base (9)..(9): 2'-deoxy-2'-fluoroguanosine
  modified_base (10)..(10): 2'-methoxyadenosine
  modified_base (11)..(11): 2'-deoxy-2'-fluorocytidine
  modified_base (12)..(12): 2'-methoxyuridine
  modified_base (13)..(13): 2'-deoxy-2'-fluoroguanosine
  modified_base (14)..(14): 2'-methoxyuridine
  modified_base (15)..(15): 2'-deoxy-2'-fluoroadenosine
  modified_base (16)..(16): 2'-methoxyguanosine
  modified_base (17)..(17): 2'-deoxy-2'-fluoroadenosine
  modified_base (18)..(18): 2'-methoxyuridine
  modified_base (19)..(19): 2'-deoxy-2'-fluorouridine
  modified_base (20)..(20): 2'-methoxyuridine
  modified_base (21)..(21): 2'-deoxy-2'-fluorouridine
  misc_feature (21)..(22): 5'-phosphorothioated
  modified_base (22)..(22): 2'-methoxyadenosine
  misc_feature (22)..(23): 5'-phosphorothioated
  modified_base (23)..(23): 2'-deoxy-2'-fluorouridine
auuccuaugacuguagauuuuau

SEQ ID NO: 47 - RNA, 27 nt, Artificial Sequence
  HPRT1_csRNA35
  modified_base (1)..(1): 2'-deoxy-2'-fluoroadenosine
  misc_feature (1)..(2): 5'-phosphorothioated
  modified_base (2)..(2): 2'-methoxyuridine
  misc_feature (2)..(3): 5'-phosphorothioated
  modified_base (3)..(3): 2'-deoxy-2'-fluorocytidine
  modified_base (4)..(4): 2'-methoxycytidine
  modified_base (5)..(5): 2'-deoxy-2'-fluoroadenosine
  modified_base (6)..(6): 2'-methoxyuridine
  modified_base (7)..(7): 2'-deoxy-2'-fluorouridine
  modified_base (8)..(8): 2'-methoxycytidine
  modified_base (9)..(9): 2'-deoxy-2'-fluorocytidine
  modified_base (10)..(10): 2'-methoxyuridine
  modified_base (11)..(11): 2'-deoxy-2'-fluoroadenosine
  modified_base (12)..(12): 2'-methoxyuridine
  modified_base (13)..(13): 2'-deoxy-2'-fluoroguanosine
  modified_base (14)..(14): 2'-methoxyadenosine
  modified_base (15)..(15): 2'-deoxy-2'-fluorocytidine
  modified_base (16)..(16): 2'-methoxyuridine
  modified_base (17)..(17): 2'-deoxy-2'-fluoroguanosine
  modified_base (18)..(18): 2'-methoxyuridine
  modified_base (19)..(19): 2'-deoxy-2'-fluoroadenosine
  modified_base (20)..(20): 2'-methoxyguanosine
  modified_base (21)..(21): 2'-deoxy-2'-fluoroadenosine
  modified_base (22)..(22): 2'-methoxyuridine
  modified_base (23)..(23): 2'-deoxy-2'-fluorouridine
  modified_base (24)..(24): 2'-methoxyuridine
  modified_base (25)..(25): 2'-deoxy-2'-fluorouridine
  misc_feature (25)..(26): 5'-phosphorothioated
  modified_base (26)..(26): 2'-methoxyadenosine
  misc_feature (26)..(27): 5'-phosphorothioated
  modified_base (27)..(27): 2'-deoxy-2'-fluorouridine
auccauuccuaugacuguagauuuuau

SEQ ID NO: 48 - RNA, 27 nt, Artificial Sequence
  HPRT1_csRNA36
  modified_base (1)..(1): 2'-deoxy-2'-fluoroadenosine
  misc_feature (1)..(2): 5'-phosphorothioated
  modified_base (2)..(2): 2'-methoxyuridine
  misc_feature (2)..(3): 5'-phosphorothioated
  modified_base (3)..(3): 2'-deoxy-2'-fluorocytidine
  modified_base (4)..(4): 2'-methoxycytidine
  modified_base (5)..(5): 2'-deoxy-2'-fluoroadenosine
  modified_base (6)..(6): 2'-methoxyuridine
  modified_base (7)..(7): 2'-deoxy-2'-fluorouridine
  modified_base (8)..(8): 2'-methoxycytidine
  modified_base (9)..(9): 2'-deoxy-2'-fluorocytidine
  modified_base (10)..(10): 2'-methoxyuridine
  modified_base (11)..(11): 2'-deoxy-2'-fluoroadenosine
  modified_base (12)..(12): 2'-methoxyuridine
  modified_base (13)..(13): 2'-deoxy-2'-fluoroguanosine
  modified_base (14)..(14): 2'-methoxyadenosine
  modified_base (15)..(15): 2'-deoxy-2'-fluorocytidine
  modified_base (16)..(16): 2'-methoxyuridine
  modified_base (17)..(17): 2'-deoxy-2'-fluoroguanosine
  modified_base (18)..(18): 2'-methoxyuridine
  modified_base (19)..(19): 2'-deoxy-2'-fluoroadenosine
  modified_base (20)..(20): 2'-methoxyguanosine
  modified_base (21)..(21): 2'-deoxy-2'-fluoroadenosine
  modified_base (22)..(22): 2'-methoxyuridine
  modified_base (23)..(23): 2'-deoxy-2'-fluorouridine
  modified_base (24)..(24): 2'-methoxyuridine
  modified_base (25)..(25): 2'-deoxy-2'-fluorouridine
  misc_feature (25)..(26): 5'-phosphorothioated
  modified_base (26)..(26): 2'-methoxyadenosine
  misc_feature (26)..(27): 5'-phosphorothioated
  modified_base (27)..(27): 2'-deoxy-2'-fluorouridine
auccauuccuaugacuguagauuuuau

SEQ ID NO: 49 - RNA, 23 nt, Artificial Sequence
  HPRT1_csRNA37
  modified_base (1)..(1): 2'-deoxy-2'-fluoroadenosine
  misc_feature (1)..(2): 5'-phosphorothioated
  modified_base (2)..(2): 2'-methoxyuridine
  misc_feature (2)..(3): 5'-phosphorothioated
  modified_base (3)..(3): 2'-deoxy-2'-fluorouridine
  modified_base (4)..(4): 2'-methoxycytidine
  modified_base (5)..(5): 2'-deoxy-2'-fluorocytidine
  modified_base (6)..(6): 2'-methoxyuridine
  modified_base (7)..(7): 2'-deoxy-2'-fluoroadenosine
  modified_base (8)..(8): 2'-methoxyuridine
  modified_base (9)..(9): 2'-deoxy-2'-fluoroguanosine
  modified_base (10)..(10): 2'-methoxyadenosine
  modified_base (11)..(11): 2'-deoxy-2'-fluorocytidine
  modified_base (12)..(12): 2'-methoxyuridine
  modified_base (13)..(13): 2'-deoxy-2'-fluoroguanosine
  modified_base (14)..(14): 2'-methoxyuridine
  modified_base (15)..(15): 2'-deoxy-2'-fluoroadenosine
  modified_base (16)..(16): 2'-methoxyguanosine
  modified_base (17)..(17): 2'-deoxy-2'-fluoroadenosine
  modified_base (18)..(18): 2'-methoxyuridine
  modified_base (19)..(19): 2'-deoxy-2'-fluorouridine
  modified_base (20)..(20): 2'-methoxyuridine
  modified_base (21)..(21): 2'-deoxy-2'-fluorouridine
  misc_feature (21)..(22): 5'-phosphorothioated
  modified_base (22)..(22): 2'-methoxyadenosine
  misc_feature (22)..(23): 5'-phosphorothioated
  modified_base (23)..(23): 2'-deoxy-2'-fluorouridine
auuccuaugacuguagauuuuau

SEQ ID NO: 50 - RNA, 27 nt, Artificial Sequence
  HPRT1_csRNA38
  modified_base (1)..(1): 2'-deoxy-2'-fluoroadenosine
  misc_feature (1)..(2): 5'-phosphorothioated
  modified_base (2)..(2): 2'-methoxyuridine
  misc_feature (2)..(3): 5'-phosphorothioated
  modified_base (3)..(3): 2'-deoxy-2'-fluorocytidine
  modified_base (4)..(4): 2'-methoxycytidine
  modified_base (5)..(5): 2'-deoxy-2'-fluoroadenosine
  modified_base (6)..(6): 2'-methoxyuridine
  modified_base (7)..(7): 2'-deoxy-2'-fluorouridine
  modified_base (8)..(8): 2'-methoxycytidine
  modified_base (9)..(9): 2'-deoxy-2'-fluorocytidine
  modified_base (10)..(10): 2'-methoxyuridine
  modified_base (11)..(11): 2'-deoxy-2'-fluoroadenosine
  modified_base (12)..(12): 2'-methoxyuridine
  modified_base (13)..(13): 2'-deoxy-2'-fluoroguanosine
  modified_base (14)..(14): 2'-methoxyadenosine
  modified_base (15)..(15): 2'-deoxy-2'-fluorocytidine
  modified_base (16)..(16): 2'-methoxyuridine
  modified_base (17)..(17): 2'-deoxy-2'-fluoroguanosine
  modified_base (18)..(18): 2'-methoxyuridine
  modified_base (19)..(19): 2'-deoxy-2'-fluoroadenosine
  modified_base (20)..(20): 2'-methoxyguanosine
  modified_base (21)..(21): 2'-deoxy-2'-fluoroadenosine
  modified_base (22)..(22): 2'-methoxyuridine
  modified_base (23)..(23): 2'-deoxy-2'-fluorouridine
  modified_base (24)..(24): 2'-methoxyuridine
  modified_base (25)..(25): 2'-deoxy-2'-fluorouridine
  misc_feature (25)..(26): 5'-phosphorothioated
  modified_base (26)..(26): 2'-methoxyadenosine
  misc_feature (26)..(27): 5'-phosphorothioated
  modified_base (27)..(27): 2'-deoxy-2'-fluorouridine
auccauuccuaugacuguagauuuuau

SEQ ID NO: 51 - RNA, 27 nt, Artificial Sequence
  HPRT1_csRNA39
  modified_base (1)..(1): 2'-deoxy-2'-fluoroadenosine
  misc_feature (1)..(2): 5'-phosphorothioated
  modified_base (2)..(2): 2'-methoxyuridine
  misc_feature (2)..(3): 5'-phosphorothioated
  modified_base (3)..(3): 2'-deoxy-2'-fluorocytidine
  modified_base (4)..(4): 2'-methoxycytidine
  modified_base (5)..(5): 2'-deoxy-2'-fluoroadenosine
  modified_base (6)..(6): 2'-methoxyuridine
  modified_base (7)..(7): 2'-deoxy-2'-fluorouridine
  modified_base (8)..(8): 2'-methoxycytidine
  modified_base (9)..(9): 2'-deoxy-2'-fluorocytidine
  modified_base (10)..(10): 2'-methoxyuridine
  modified_base (11)..(11): 2'-deoxy-2'-fluoroadenosine
  modified_base (12)..(12): 2'-methoxyuridine
  modified_base (13)..(13): 2'-deoxy-2'-fluoroguanosine
  modified_base (14)..(14): 2'-methoxyadenosine
  modified_base (15)..(15): 2'-deoxy-2'-fluorocytidine
  modified_base (16)..(16): 2'-methoxyuridine
  modified_base (17)..(17): 2'-deoxy-2'-fluoroguanosine
  modified_base (18)..(18): 2'-methoxyuridine
  modified_base (19)..(19): 2'-deoxy-2'-fluoroadenosine
  modified_base (20)..(20): 2'-methoxyguanosine
  modified_base (21)..(21): 2'-deoxy-2'-fluoroadenosine
  modified_base (22)..(22): 2'-methoxyuridine
  modified_base (23)..(23): 2'-deoxy-2'-fluorouridine
  modified_base (24)..(24): 2'-methoxyuridine
  modified_base (25)..(25): 2'-deoxy-2'-fluorouridine
  misc_feature (25)..(26): 5'-phosphorothioated
  modified_base (26)..(26): 2'-methoxyadenosine
  misc_feature (26)..(27): 5'-phosphorothioated
  modified_base (27)..(27): 2'-deoxy-2'-fluorouridine
auccauuccuaugacuguagauuuuau

SEQ ID NO: 52 - RNA, 27 nt, Artificial Sequence
  HPRT1_csRNA40
  modified_base (1)..(1): 2'-deoxy-2'-fluoroadenosine
  misc_feature (1)..(2): 5'-phosphorothioated
  modified_base (2)..(2): 2'-methoxyuridine
  misc_feature (2)..(3): 5'-phosphorothioated
  modified_base (3)..(3): 2'-deoxy-2'-fluorocytidine
  modified_base (4)..(4): 2'-methoxycytidine
  modified_base (5)..(5): 2'-deoxy-2'-fluoroadenosine
  modified_base (6)..(6): 2'-methoxyuridine
  modified_base (7)..(7): 2'-deoxy-2'-fluorouridine
  modified_base (8)..(8): 2'-methoxycytidine
  modified_base (9)..(9): 2'-deoxy-2'-fluorocytidine
  modified_base (10)..(10): 2'-methoxyuridine
  modified_base (11)..(11): 2'-deoxy-2'-fluoroadenosine
  modified_base (12)..(12): 2'-methoxyuridine
  modified_base (13)..(13): 2'-deoxy-2'-fluoroguanosine
  modified_base (14)..(14): 2'-methoxyadenosine
  modified_base (15)..(15): 2'-deoxy-2'-fluorocytidine
  modified_base (16)..(16): 2'-methoxyuridine
  modified_base (17)..(17): 2'-deoxy-2'-fluoroguanosine
  modified_base (18)..(18): 2'-methoxyuridine
  modified_base (19)..(19): 2'-deoxy-2'-fluoroadenosine
  modified_base (20)..(20): 2'-methoxyguanosine
  modified_base (21)..(21): 2'-deoxy-2'-fluoroadenosine
  modified_base (22)..(22): 2'-methoxyuridine
  modified_base (23)..(23): 2'-deoxy-2'-fluorouridine
  modified_base (24)..(24): 2'-methoxyuridine
  modified_base (25)..(25): 2'-deoxy-2'-fluorouridine
  misc_feature (25)..(26): 5'-phosphorothioated
  modified_base (26)..(26): 2'-methoxyadenosine
  misc_feature (26)..(27): 5'-phosphorothioated
  modified_base (27)..(27): 2'-deoxy-2'-fluorouridine
auccauuccuaugacuguagauuuuau

SEQ ID NO: 53 - RNA, 27 nt, Artificial Sequence
  HPRT1_csRNA41
  modified_base (1)..(1): 2'-deoxy-2'-fluoroguanosine
  misc_feature (1)..(2): 5'-phosphorothioated
  modified_base (2)..(2): 2'-methoxyguanosine
  misc_feature (2)..(3): 5'-phosphorothioated
  modified_base (3)..(3): 2'-deoxy-2'-fluoroadenosine
  modified_base (4)..(4): 2'-methoxyuridine
  modified_base (5)..(5): 2'-deoxy-2'-fluoroadenosine
  modified_base (6)..(6): 2'-methoxyuridine
  modified_base (7)..(7): 2'-deoxy-2'-fluoroadenosine
  modified_base (8)..(8): 2'-methoxyadenosine
  modified_base (9)..(9): 2'-deoxy-2'-fluoroguanosine
  modified_base (10)..(10): 2'-methoxycytidine
  modified_base (11)..(11): 2'-deoxy-2'-fluorocytidine
  modified_base (12)..(12): 2'-methoxyadenosine
  modified_base (13)..(13): 2'-deoxy-2'-fluoroguanosine
  modified_base (14)..(14): 2'-methoxyadenosine
  modified_base (15)..(15): 2'-deoxy-2'-fluorocytidine
  modified_base (16)..(16): 2'-methoxyuridine
  modified_base (17)..(17): 2'-deoxy-2'-fluorouridine
  modified_base (18)..(18): 2'-methoxyuridine
  modified_base (19)..(19): 2'-deoxy-2'-fluoroguanosine
  modified_base (20)..(20): 2'-methoxyuridine
  modified_base (21)..(21): 2'-deoxy-2'-fluorouridine
  modified_base (22)..(22): 2'-methoxyguanosine
  modified_base (23)..(23): 2'-deoxy-2'-fluoroguanosine
  modified_base (24)..(24): 2'-methoxyadenosine
  modified_base (25)..(25): 2'-deoxy-2'-fluorouridine
  modified_base (26)..(26): 2'-methoxyuridine
  modified_base (27)..(27): 2'-deoxy-2'-fluorouridine
ggauauaagccagacuuuguuggauuu

SEQ ID NO: 54 - RNA, 27 nt, Artificial Sequence
  HPRT1_csRNA42
  modified_base (1)..(1): 2'-deoxy-2'-fluoroadenosine
  misc_feature (1)..(2): 5'-phosphorothioated
  modified_base (2)..(2): 2'-methoxyuridine
  misc_feature (2)..(3): 5'-phosphorothioated
  modified_base (3)..(3): 2'-deoxy-2'-fluorocytidine
  modified_base (4)..(4): 2'-methoxycytidine
  modified_base (5)..(5): 2'-deoxy-2'-fluoroadenosine
  modified_base (6)..(6): 2'-methoxyuridine
  modified_base (7)..(7): 2'-deoxy-2'-fluorouridine
  modified_base (8)..(8): 2'-methoxycytidine
  modified_base (9)..(9): 2'-deoxy-2'-fluorocytidine
  modified_base (10)..(10): 2'-methoxyuridine
  modified_base (11)..(11): 2'-deoxy-2'-fluoroadenosine
  modified_base (12)..(12): 2'-methoxyuridine
  modified_base (13)..(13): 2'-deoxy-2'-fluoroguanosine
  modified_base (14)..(14): 2'-methoxyadenosine
  modified_base (15)..(15): 2'-deoxy-2'-fluorocytidine
  modified_base (16)..(16): 2'-methoxyuridine
  modified_base (17)..(17): 2'-deoxy-2'-fluoroguanosine
  modified_base (18)..(18): 2'-methoxyuridine
  modified_base (19)..(19): 2'-deoxy-2'-fluoroadenosine
  modified_base (20)..(20): 2'-methoxyguanosine
  modified_base (21)..(21): 2'-deoxy-2'-fluoroadenosine
  modified_base (22)..(22): 2'-methoxyuridine
  modified_base (23)..(23): 2'-deoxy-2'-fluorouridine
  modified_base (24)..(24): 2'-methoxyuridine
  modified_base (25)..(25): 2'-deoxy-2'-fluorouridine
  misc_feature (25)..(26): 5'-phosphorothioated
  modified_base (26)..(26): 2'-methoxyadenosine
  misc_feature (26)..(27): 5'-phosphorothioated
  modified_base (27)..(27): 2'-deoxy-2'-fluorouridine
auccauuccuaugacuguagauuuuau

SEQ ID NO: 55 - RNA, 27 nt, Artificial Sequence
  HPRT1_csRNA43
  modified_base (1)..(1): 2'-deoxy-2'-fluoroadenosine
  misc_feature (1)..(2): 5'-phosphorothioated
  modified_base (2)..(2): 2'-methoxyuridine
  misc_feature (2)..(3): 5'-phosphorothioated
  modified_base (3)..(3): 2'-deoxy-2'-fluorocytidine
  modified_base (4)..(4): 2'-methoxycytidine
  modified_base (5)..(5): 2'-deoxy-2'-fluoroadenosine
  modified_base (6)..(6): 2'-methoxyuridine
  modified_base (7)..(7): 2'-deoxy-2'-fluorouridine
  modified_base (8)..(8): 2'-methoxycytidine
  modified_base (9)..(9): 2'-deoxy-2'-fluorocytidine
  modified_base (10)..(10): 2'-methoxyuridine
  modified_base (11)..(11): 2'-deoxy-2'-fluoroadenosine
  modified_base (12)..(12): 2'-methoxyuridine
  modified_base (13)..(13): 2'-deoxy-2'-fluoroguanosine
  modified_base (14)..(14): 2'-methoxyadenosine
  modified_base (15)..(15): 2'-deoxy-2'-fluorocytidine
  modified_base (16)..(16): 2'-methoxyuridine
  modified_base (17)..(17): 2'-deoxy-2'-fluoroguanosine
  modified_base (18)..(18): 2'-methoxyuridine
  modified_base (19)..(19): 2'-deoxy-2'-fluoroadenosine
  modified_base (20)..(20): 2'-methoxyguanosine
  modified_base (21)..(21): 2'-deoxy-2'-fluoroadenosine
  modified_base (22)..(22): 2'-methoxyuridine
  modified_base (23)..(23): 2'-deoxy-2'-fluorouridine
  modified_base (24)..(24): 2'-methoxyuridine
  modified_base (25)..(25): 2'-deoxy-2'-fluorouridine
  misc_feature (25)..(26): 5'-phosphorothioated
  modified_base (26)..(26): 2'-methoxyadenosine
  misc_feature (26)..(27): 5'-phosphorothioated
  modified_base (27)..(27): 2'-deoxy-2'-fluorouridine
auccauuccuaugacuguagauuuuau

SEQ ID NO: 56 - RNA, 27 nt, Artificial Sequence
  HPRT1_csRNA44
  modified_base (1)..(1): 2'-deoxy-2'-fluoroadenosine
  misc_feature (1)..(2): 5'-phosphorothioated
  modified_base (2)..(2): 2'-methoxyuridine
  misc_feature (2)..(3): 5'-phosphorothioated
  modified_base (3)..(3): 2'-deoxy-2'-fluorocytidine
  modified_base (4)..(4): 2'-methoxycytidine
  modified_base (5)..(5): 2'-deoxy-2'-fluoroadenosine
  modified_base (6)..(6): 2'-methoxyuridine
  modified_base (7)..(7): 2'-deoxy-2'-fluorouridine
  modified_base (8)..(8): 2'-methoxycytidine
  modified_base (9)..(9): 2'-deoxy-2'-fluorocytidine
  modified_base (10)..(10): 2'-methoxyuridine
  modified_base (11)..(11): 2'-deoxy-2'-fluoroadenosine
  modified_base (12)..(12): 2'-methoxyuridine
  modified_base (13)..(13): 2'-deoxy-2'-fluoroguanosine
  modified_base (14)..(14): 2'-methoxyadenosine
  modified_base (15)..(15): 2'-deoxy-2'-fluorocytidine
  modified_base (16)..(16): 2'-methoxyuridine
  modified_base (17)..(17): 2'-deoxy-2'-fluoroguanosine
  modified_base (18)..(18): 2'-methoxyuridine
  modified_base (19)..(19): 2'-deoxy-2'-fluoroadenosine
  modified_base (20)..(20): 2'-methoxyguanosine
  modified_base (21)..(21): 2'-deoxy-2'-fluoroadenosine
  modified_base (22)..(22): 2'-methoxyuridine
  modified_base (23)..(23): 2'-deoxy-2'-fluorouridine
  modified_base (24)..(24): 2'-methoxyuridine
  modified_base (25)..(25): 2'-deoxy-2'-fluorouridine
  misc_feature (25)..(26): 5'-phosphorothioated
  modified_base (26)..(26): 2'-methoxyadenosine
  misc_feature (26)..(27): 5'-phosphorothioated
  modified_base (27)..(27): 2'-deoxy-2'-fluorouridine
auccauuccuaugacuguagauuuuau

SEQ ID NO: 57 - RNA, 19 nt, Artificial Sequence
  PTEN_ssRNA1
  modified_base (1)..(1): 2'-deoxy-2'-fluoroadenosine
  misc_feature (1)..(2): 5'-phosphorothioated
  modified_base (2)..(2): 2'-methoxycytidine
  misc_feature (2)..(3): 5'-phosphorothioated
  modified_base (3)..(3): 2'-deoxy-2'-fluorocytidine
  modified_base (4)..(4): 2'-methoxyuridine
  modified_base (5)..(5): 2'-deoxy-2'-fluoroguanosine
  modified_base (6)..(6): 2'-methoxyadenosine
  modified_base (7)..(7): 2'-deoxy-2'-fluorouridine
  modified_base (8)..(8): 2'-methoxycytidine
  modified_base (9)..(9): 2'-deoxy-2'-fluoroadenosine
  modified_base (10)..(10): 2'-methoxyuridine
  modified_base (11)..(11): 2'-deoxy-2'-fluorouridine
  modified_base (12)..(12): 2'-methoxyadenosine
  modified_base (13)..(13): 2'-deoxy-2'-fluorouridine
  modified_base (14)..(14): 2'-methoxyadenosine
  modified_base (15)..(15): 2'-deoxy-2'-fluoroguanosine
  modified_base (16)..(16): 2'-methoxyadenosine
  modified_base (17)..(17): 2'-deoxy-2'-fluorouridine
  misc_feature (17)..(18): 5'-phosphorothioated
  modified_base (18)..(18): 2'-methoxyadenosine
  misc_feature (18)..(19): 5'-phosphorothioated
  modified_base (19)..(19): 2'-deoxy-2'-fluoroadenosine
accugaucauuauagauaa

SEQ ID NO: 58 - RNA, 27 nt, Artificial Sequence
  PTEN_ssRNA2
  modified_base (1)..(1): 2'-deoxy-2'-fluoroguanosine
  misc_feature (1)..(2): 5'-phosphorothioated
  modified_base (2)..(2): 2'-methoxyadenosine
  misc_feature (2)..(3): 5'-phosphorothioated
  modified_base (3)..(3): 2'-deoxy-2'-fluorocytidine
  modified_base (4)..(4): 2'-methoxyadenosine
  modified_base (5)..(5): 2'-deoxy-2'-fluoroadenosine
  modified_base (6)..(6): 2'-methoxyuridine
  modified_base (7)..(7): 2'-deoxy-2'-fluoroguanosine
  modified_base (8)..(8): 2'-methoxyadenosine
  modified_base (9)..(9): 2'-deoxy-2'-fluoroadenosine
  modified_base (10)..(10): 2'-methoxycytidine
  modified_base (11)..(11): 2'-deoxy-2'-fluorocytidine
  modified_base (12)..(12): 2'-methoxyuridine
  modified_base (13)..(13): 2'-deoxy-2'-fluoroguanosine
  modified_base (14)..(14): 2'-methoxyadenosine
  modified_base (15)..(15): 2'-deoxy-2'-fluorouridine
  modified_base (16)..(16): 2'-methoxycytidine
  modified_base (17)..(17): 2'-deoxy-2'-fluoroadenosine
  modified_base (18)..(18): 2'-methoxyuridine
  modified_base (19)..(19): 2'-deoxy-2'-fluorouridine
  modified_base (20)..(20): 2'-methoxyadenosine
  modified_base (21)..(21): 2'-deoxy-2'-fluorouridine
  modified_base (22)..(22): 2'-methoxyadenosine
  modified_base (23)..(23): 2'-deoxy-2'-fluoroguanosine
  modified_base (24)..(24): 2'-methoxyadenosine
  modified_base (25)..(25): 2'-deoxy-2'-fluorouridine
  misc_feature (25)..(26): 5'-phosphorothioated
  modified_base (26)..(26): 2'-methoxyadenosine
  misc_feature (26)..(27): 5'-phosphorothioated
  modified_base (27)..(27): 2'-deoxy-2'-fluoroadenosine
gacaaugaaccugaucauuauagauaa

SEQ ID NO: 59 - RNA, 21 nt, Artificial Sequence
  PTEN_asRNA1
  modified_base (1)..(1): 2'-methoxyuridine
  misc_feature (1)..(2): 5'-phosphorothioated
  modified_base (2)..(2): 2'-deoxy-2'-fluorouridine
  misc_feature (2)..(3): 5'-phosphorothioated
  modified_base (3)..(3): 2'-methoxyadenosine
  modified_base (4)..(4): 2'-deoxy-2'-fluorouridine
  modified_base (5)..(5): 2'-methoxycytidine
  modified_base (6)..(6): 2'-deoxy-2'-fluorouridine
  modified_base (7)..(7): 2'-methoxyadenosine
  modified_base (8)..(8): 2'-deoxy-2'-fluorouridine
  modified_base (9)..(9): 2'-methoxyadenosine
  modified_base (10)..(10): 2'-deoxy-2'-fluoroadenosine
  modified_base (11)..(11): 2'-methoxyuridine
  modified_base (12)..(12): 2'-deoxy-2'-fluoroguanosine
  modified_base (13)..(13): 2'-methoxyadenosine
  modified_base (14)..(14): 2'-deoxy-2'-fluorouridine
  modified_base (15)..(15): 2'-methoxycytidine
  modified_base (16)..(16): 2'-deoxy-2'-fluoroadenosine
  modified_base (17)..(17): 2'-methoxyguanosine
  modified_base (18)..(18): 2'-deoxy-2'-fluoroguanosine
  modified_base (19)..(19): 2'-methoxyuridine
  misc_feature (19)..(20): 5'-phosphorothioated
  modified_base (20)..(20): 2'-deoxy-2'-fluoroadenosine
  misc_feature (20)..(21): 5'-phosphorothioated
  modified_base (21)..(21): 2'-methoxyadenosine
uuaucuauaaugaucagguaa

SEQ ID NO: 60 - RNA, 21 nt, Artificial Sequence
  PTEN_asRNA2
  modified_base (1)..(1): 2'-methoxyuridine
  misc_feature (1)..(2): 5'-phosphorothioated
  modified_base (2)..(2): 2'-deoxy-2'-fluorouridine
  misc_feature (2)..(3): 5'-phosphorothioated
  modified_base (3)..(3): 2'-methoxyadenosine
  modified_base (4)..(4): 2'-deoxy-2'-fluorouridine
  modified_base (5)..(5): 2'-methoxycytidine
  modified_base (6)..(6): 2'-deoxy-2'-fluorouridine
  modified_base (7)..(7): 2'-methoxyadenosine
  modified_base (8)..(8): 2'-deoxy-2'-fluorouridine
  modified_base (9)..(9): 2'-methoxyadenosine
  modified_base (10)..(10): 2'-deoxy-2'-fluoroadenosine
  modified_base (11)..(11): 2'-methoxyuridine
  modified_base (12)..(12): 2'-deoxy-2'-fluoroguanosine
  modified_base (13)..(13): 2'-methoxyadenosine
  modified_base (14)..(14): 2'-deoxy-2'-fluorouridine
  modified_base (15)..(15): 2'-methoxycytidine
  modified_base (16)..(16): 2'-deoxy-2'-fluoroadenosine
  modified_base (17)..(17): 2'-methoxyguanosine
  modified_base (18)..(18): 2'-deoxy-2'-fluoroguanosine
  modified_base (19)..(19): 2'-methoxyuridine
  misc_feature (19)..(20): 5'-phosphorothioated
  modified_base (20)..(20): 2'-deoxy-2'-fluorouridine
  misc_feature (20)..(21): 5'-phosphorothioated
  modified_base (21)..(21): 2'-methoxycytidine
uuaucuauaaugaucagguuc

SEQ ID NO: 61 - RNA, 27 nt, Artificial Sequence
  PTEN_csRNA1
  modified_base (1)..(1): 2'-deoxy-2'-fluoroguanosine
  misc_feature (1)..(2): 5'-phosphorothioated
  modified_base (2)..(2): 2'-methoxyadenosine
  misc_feature (2)..(3): 5'-phosphorothioated
  modified_base (3)..(3): 2'-deoxy-2'-fluorocytidine
  modified_base (4)..(4): 2'-methoxyadenosine
  modified_base (5)..(5): 2'-deoxy-2'-fluoroadenosine
  modified_base (6)..(6): 2'-methoxyuridine
  modified_base (7)..(7): 2'-deoxy-2'-fluoroguanosine
  modified_base (8)..(8): 2'-methoxyadenosine
  modified_base (9)..(9): 2'-deoxy-2'-fluoroadenosine
  modified_base (10)..(10): 2'-methoxycytidine
  modified_base (11)..(11): 2'-deoxy-2'-fluorocytidine
  modified_base (12)..(12): 2'-methoxyuridine
  modified_base (13)..(13): 2'-deoxy-2'-fluoroguanosine
  modified_base (14)..(14): 2'-methoxyadenosine
  modified_base (15)..(15): 2'-deoxy-2'-fluorouridine
  modified_base (16)..(16): 2'-methoxycytidine
  modified_base (17)..(17): 2'-deoxy-2'-fluoroadenosine
  modified_base (18)..(18): 2'-methoxyuridine
  modified_base (19)..(19): 2'-deoxy-2'-fluorouridine
  modified_base (20)..(20): 2'-methoxyadenosine
  modified_base (21)..(21): 2'-deoxy-2'-fluorouridine
  modified_base (22)..(22): 2'-methoxyadenosine
  modified_base (23)..(23): 2'-deoxy-2'-fluoroguanosine
  modified_base (24)..(24): 2'-methoxyadenosine
  modified_base (25)..(25): 2'-deoxy-2'-fluorouridine
  misc_feature (25)..(26): 5'-phosphorothioated
  modified_base (26)..(26): 2'-methoxyadenosine
  misc_feature (26)..(27): 5'-phosphorothioated
  modified_base (27)..(27): 2'-deoxy-2'-fluoroadenosine
gacaaugaaccugaucauuauagauaa

SEQ ID NO: 62 - RNA, 21 nt, Artificial Sequence
  Factor9_ssRNA1
  modified_base (1)..(1): 2'-deoxy-2'-fluorouridine
  misc_feature (1)..(2): 5'-phosphorothioated
  modified_base (2)..(2): 2'-methoxyguanosine
  misc_feature (2)..(3): 5'-phosphorothioated
  modified_base (3)..(3): 2'-deoxy-2'-fluoroguanosine
  modified_base (4)..(4): 2'-methoxyadenosine
  modified_base (5)..(5): 2'-deoxy-2'-fluoroadenosine
  modified_base (6)..(6): 2'-methoxyguanosine
  modified_base (7)..(7): 2'-deoxy-2'-fluorocytidine
  modified_base (8)..(8): 2'-methoxyadenosine
  modified_base (9)..(9): 2'-deoxy-2'-fluoroguanosine
  modified_base (10)..(10): 2'-deoxy-2'-fluorouridine
  modified_base (11)..(11): 2'-deoxy-2'-fluoroadenosine
  modified_base (12)..(12): 2'-methoxyuridine
  modified_base (13)..(13): 2'-deoxy-2'-fluoroguanosine
  modified_base (14)..(14): 2'-methoxyuridine
  modified_base (15)..(15): 2'-deoxy-2'-fluorouridine
  modified_base (16)..(16): 2'-methoxyguanosine
  modified_base (17)..(17): 2'-deoxy-2'-fluoroadenosine
  modified_base (18)..(18): 2'-methoxyuridine
  modified_base (19)..(19): 2'-deoxy-2'-fluoroguanosine
  modified_base (20)..(20): 2'-methoxyguanosine
  modified_base (21)..(21): 2'-deoxy-2'-fluoroadenosine
uggaagcaguauguugaugga

SEQ ID NO: 63 - RNA, 27 nt, Artificial Sequence
  Factor9_ssRNA2
  modified_base (1)..(1): 2'-deoxy-2'-fluoroguanosine
  misc_feature (1)..(2): 5'-phosphorothioated
  modified_base (2)..(2): 2'-methoxyadenosine
  misc_feature (2)..(3): 5'-phosphorothioated
  modified_base (3)..(3): 2'-deoxy-2'-fluoroadenosine
  modified_base (4)..(4): 2'-methoxyuridine
  modified_base (5)..(5): 2'-deoxy-2'-fluorouridine
  modified_base (6)..(6): 2'-methoxyuridine
  modified_base (7)..(7): 2'-deoxy-2'-fluorouridine
  modified_base (8)..(8): 2'-methoxyguanosine
  modified_base (9)..(9): 2'-deoxy-2'-fluoroguanosine
  modified_base (10)..(10): 2'-methoxyadenosine
  modified_base (11)..(11): 2'-deoxy-2'-fluoroadenosine
  modified_base (12)..(12): 2'-methoxyguanosine
  modified_base (13)..(13): 2'-deoxy-2'-fluorocytidine
  modified_base (14)..(14): 2'-methoxyadenosine
  modified_base (15)..(15): 2'-deoxy-2'-fluoroguanosine
  modified_base (16)..(16): 2'-deoxy-2'-fluorouridine
  modified_base (17)..(17): 2'-deoxy-2'-fluoroadenosine
  modified_base (18)..(18): 2'-methoxyuridine
  modified_base (19)..(19): 2'-deoxy-2'-fluoroguanosine
  modified_base (20)..(20): 2'-methoxyuridine
  modified_base (21)..(21): 2'-deoxy-2'-fluorouridine
  modified_base (22)..(22): 2'-methoxyguanosine
  modified_base (23)..(23): 2'-deoxy-2'-fluoroadenosine
  modified_base (24)..(24): 2'-methoxyuridine
  modified_base (25)..(25): 2'-deoxy-2'-fluoroguanosine
  modified_base (26)..(26): 2'-methoxyguanosine
  modified_base (27)..(27): 2'-deoxy-2'-fluoroadenosine
gaauuuuggaagcaguauguugaugga

SEQ ID NO: 64 - RNA, 23 nt, Artificial Sequence
  Factor9_asRNA1
  modified_base (1)..(1): 2'-methoxyuridine
  misc_feature (1)..(2): 5'-phosphorothioated
  modified_base (2)..(2): 2'-deoxy-2'-fluorocytidine
  misc_feature (2)..(3): 5'-phosphorothioated
  modified_base (3)..(3): 2'-methoxycytidine
  modified_base (4)..(4): 2'-deoxy-2'-fluoroadenosine
  modified_base (5)..(5): 2'-methoxyuridine
  modified_base (6)..(6): 2'-deoxy-2'-fluorocytidine
  modified_base (7)..(7): 2'-methoxyadenosine
  modified_base (8)..(8): 2'-deoxy-2'-fluoroadenosine
  modified_base (9)..(9): 2'-methoxycytidine
  modified_base (10)..(10): 2'-deoxy-2'-fluoroadenosine
  modified_base (11)..(11): 2'-methoxyuridine
  modified_base (12)..(12): 2'-methoxyadenosine
  modified_base (13)..(13): 2'-methoxycytidine
  modified_base (14)..(14): 2'-deoxy-2'-fluorouridine
  modified_base (15)..(15): 2'-methoxyguanosine
  modified_base (16)..(16): 2'-deoxy-2'-fluorocytidine
  modified_base (17)..(17): 2'-methoxyuridine
  modified_base (18)..(18): 2'-deoxy-2'-fluorouridine
  modified_base (19)..(19): 2'-methoxycytidine
  modified_base (20)..(20): 2'-deoxy-2'-fluorocytidine
  modified_base (21)..(21): 2'-methoxyadenosine
  misc_feature (21)..(22): 5'-phosphorothioated
  modified_base (22)..(22): 2'-methoxyadenosine
  misc_feature (22)..(23): 5'-phosphorothioated
  modified_base (23)..(23): 2'-methoxyadenosine
uccaucaacauacugcuuccaaa

SEQ ID NO: 65 - RNA, 21 nt, Artificial Sequence
  Factor9_asRNA2
  modified_base (1)..(1): 2'-methoxyuridine
  misc_feature (1)..(2): 5'-phosphorothioated
  modified_base (2)..(2): 2'-deoxy-2'-fluorocytidine
  misc_feature (2)..(3): 5'-phosphorothioated
  modified_base (3)..(3): 2'-methoxycytidine
  modified_base (4)..(4): 2'-deoxy-2'-fluoroadenosine
  modified_base (5)..(5): 2'-methoxyuridine
  modified_base (6)..(6): 2'-deoxy-2'-fluorocytidine
  modified_base (7)..(7): 2'-methoxyadenosine
  modified_base (8)..(8): 2'-deoxy-2'-fluoroadenosine
  modified_base (9)..(9): 2'-methoxycytidine
  modified_base (10)..(10): 2'-deoxy-2'-fluoroadenosine
  modified_base (11)..(11): 2'-methoxyuridine
  modified_base (12)..(12): 2'-methoxyadenosine
  modified_base (13)..(13): 2'-methoxycytidine
  modified_base (14)..(14): 2'-deoxy-2'-fluorouridine
  modified_base (15)..(15): 2'-methoxyguanosine
  modified_base (16)..(16): 2'-deoxy-2'-fluorocytidine
  modified_base (17)..(17): 2'-methoxyuridine
  modified_base (18)..(18): 2'-deoxy-2'-fluorouridine
  modified_base (19)..(19): 2'-methoxycytidine
  misc_feature (19)..(20): 5'-phosphorothioated
  modified_base (20)..(20): 2'-deoxy-2'-fluorocytidine
  misc_feature (20)..(21): 5'-phosphorothioated
  modified_base (21)..(21): 2'-methoxyadenosine
uccaucaacauacugcuucca

SEQ ID NO: 66 - RNA, 27 nt, Artificial Sequence
  Factor9_csRNA1
  modified_base (1)..(1): 2'-deoxy-2'-fluoroguanosine
  misc_feature (1)..(2): 5'-phosphorothioated
  modified_base (2)..(2): 2'-methoxyadenosine
  misc_feature (2)..(3): 5'-phosphorothioated
  modified_base (3)..(3): 2'-deoxy-2'-fluoroadenosine
  modified_base (4)..(4): 2'-methoxyuridine
  modified_base (5)..(5): 2'-deoxy-2'-fluorouridine
  modified_base (6)..(6): 2'-methoxyuridine
  modified_base (7)..(7): 2'-deoxy-2'-fluorouridine
  modified_base (8)..(8): 2'-methoxyguanosine
  modified_base (9)..(9): 2'-deoxy-2'-fluoroguanosine
  modified_base (10)..(10): 2'-methoxyadenosine
  modified_base (11)..(11): 2'-deoxy-2'-fluoroadenosine
  modified_base (12)..(12): 2'-methoxyguanosine
  modified_base (13)..(13): 2'-deoxy-2'-fluorocytidine
  modified_base (14)..(14): 2'-methoxyadenosine
  modified_base (15)..(15): 2'-deoxy-2'-fluoroguanosine
  modified_base (16)..(16): 2'-deoxy-2'-fluorouridine
  modified_base (17)..(17): 2'-deoxy-2'-fluoroadenosine
  modified_base (18)..(18): 2'-methoxyuridine
  modified_base (19)..(19): 2'-deoxy-2'-fluoroguanosine
  modified_base (20)..(20): 2'-methoxyuridine
  modified_base (21)..(21): 2'-deoxy-2'-fluorouridine
  modified_base (22)..(22): 2'-methoxyguanosine
  modified_base (23)..(23): 2'-deoxy-2'-fluoroadenosine
  modified_base (24)..(24): 2'-methoxyuridine
  modified_base (25)..(25): 2'-deoxy-2'-fluoroguanosine
  modified_base (26)..(26): 2'-methoxyguanosine
  modified_base (27)..(27): 2'-deoxy-2'-fluoroadenosine
gaauuuuggaagcaguauguugaugga

SEQ ID NO: 67 - RNA, 21 nt, Artificial Sequence
  B2M_ssRNA1
  modified_base (1)..(1): 2'-deoxy-2'-fluoroadenosine
  modified_base (2)..(2): 2'-methoxyguanosine
  modified_base (3)..(3): 2'-deoxy-2'-fluoroguanosine
  modified_base (4)..(4): 2'-methoxyadenosine
  modified_base (5)..(5): 2'-deoxy-2'-fluorocytidine
  modified_base (6)..(6): 2'-methoxyuridine
  modified_base (7)..(7): 2'-deoxy-2'-fluoroguanosine
  modified_base (8)..(8): 2'-methoxyguanosine
  modified_base (9)..(9): 2'-deoxy-2'-fluorouridine
  modified_base (10)..(10): 2'-methoxycytidine
  modified_base (11)..(11): 2'-deoxy-2'-fluorouridine
  modified_base (12)..(12): 2'-deoxy-2'-fluorouridine
  modified_base (13)..(13): 2'-methoxyuridine
  modified_base (14)..(14): 2'-deoxy-2'-fluorocytidine
  modified_base (15)..(15): 2'-methoxyuridine
  modified_base (16)..(16): 2'-deoxy-2'-fluoroadenosine
  modified_base (17)..(17): 2'-methoxyuridine
  modified_base (18)..(18): 2'-deoxy-2'-fluoroadenosine
  modified_base (19)..(19): 2'-methoxyuridine
  misc_feature (19)..(20): 5'-phosphorothioated
  modified_base (20)..(20): 2'-deoxy-2'-fluorocytidine
  misc_feature (20)..(21): 5'-phosphorothioated
  modified_base (21)..(21): 2'-methoxyuridine
aggacuggucuuucuauaucu

SEQ ID NO: 68 - RNA, 25 nt, Artificial Sequence
  BM2_ssRNA2
  modified_base (1)..(1): 2'-deoxy-2'-fluoroadenosine
  modified_base (2)..(2): 2'-methoxyguanosine
  modified_base (3)..(3): 2'-deoxy-2'-fluorocytidine
  modified_base (4)..(4): 2'-methoxyadenosine
  modified_base (5)..(5): 2'-deoxy-2'-fluoroadenosine
  modified_base (6)..(6): 2'-methoxyguanosine
  modified_base (7)..(7): 2'-deoxy-2'-fluoroguanosine
  modified_base (8)..(8): 2'-methoxyadenosine
  modified_base (9)..(9): 2'-deoxy-2'-fluorocytidine
  modified_base (10)..(10): 2'-methoxyuridine
  modified_base (11)..(11): 2'-deoxy-2'-fluoroguanosine
  modified_base (12)..(12): 2'-methoxyguanosine
  modified_base (13)..(13): 2'-deoxy-2'-fluorouridine
  modified_base (14)..(14): 2'-methoxycytidine
  modified_base (15)..(15): 2'-deoxy-2'-fluorouridine
  modified_base (16)..(16): 2'-deoxy-2'-fluorouridine
  modified_base (17)..(17): 2'-methoxyuridine
  modified_base (18)..(18): 2'-deoxy-2'-fluorocytidine
  modified_base (19)..(19): 2'-methoxyuridine
  modified_base (20)..(20): 2'-deoxy-2'-fluoroadenosine
  modified_base (21)..(21): 2'-methoxyuridine
  modified_base (22)..(22): 2'-deoxy-2'-fluoroadenosine
  modified_base (23)..(23): 2'-methoxyuridine
  misc_feature (23)..(24): 5'-phosphorothioated
  modified_base (24)..(24): 2'-deoxy-2'-fluorocytidine
  misc_feature (24)..(25): 5'-phosphorothioated
  modified_base (25)..(25): 2'-methoxyuridine
agcaaggacuggucuuucuauaucu

SEQ ID NO: 69 - RNA, 21 nt, Artificial Sequence
  B2M_asRNA1
  modified_base (1)..(1): 2'-deoxy-2'-fluoroadenosine
  misc_feature (1)..(2): 5'-phosphorothioated
  modified_base (2)..(2): 2'-methoxyguanosine
  misc_feature (2)..(3): 5'-phosphorothioated
  modified_base (3)..(3): 2'-deoxy-2'-fluoroadenosine
  modified_base (4)..(4): 2'-methoxyuridine
  modified_base (5)..(5): 2'-deoxy-2'-fluoroadenosine
  modified_base (6)..(6): 2'-methoxyuridine
  modified_base (7)..(7): 2'-deoxy-2'-fluoroadenosine
  modified_base (8)..(8): 2'-methoxyguanosine
  modified_base (9)..(9): 2'-deoxy-2'-fluoroadenosine
  modified_base (10)..(10): 2'-methoxyadenosine
  modified_base (11)..(11): 2'-methoxyadenosine
  modified_base (12)..(12): 2'-deoxy-2'-fluoroguanosine
  modified_base (13)..(13): 2'-methoxyadenosine
  modified_base (14)..(14): 2'-deoxy-2'-fluorocytidine
  modified_base (15)..(15): 2'-methoxycytidine
  modified_base (16)..(16): 2'-deoxy-2'-fluoroadenosine
  modified_base (17)..(17): 2'-methoxyguanosine
  modified_base (18)..(18): 2'-deoxy-2'-fluorouridine
  modified_base (19)..(19): 2'-methoxycytidine
  misc_feature (19)..(20): 5'-phosphorothioated
  modified_base (20)..(20): 2'-deoxy-2'-fluorocytidine
  misc_feature (20)..(21): 5'-phosphorothioated
  modified_base (21)..(21): 2'-methoxyuridine
agauauagaaagaccaguccu

SEQ ID NO: 70 - RNA, 25 nt, Artificial Sequence
  B2M_csRNA1
  modified_base (1)..(1): 2'-deoxy-2'-fluoroadenosine
  modified_base (2)..(2): 2'-methoxyguanosine
  modified_base (3)..(3): 2'-deoxy-2'-fluorocytidine
  modified_base (4)..(4): 2'-methoxyadenosine
  modified_base (5)..(5): 2'-deoxy-2'-fluoroadenosine
  modified_base (6)..(6): 2'-methoxyguanosine
  modified_base (7)..(7): 2'-deoxy-2'-fluoroguanosine
  modified_base (8)..(8): 2'-methoxyadenosine
  modified_base (9)..(9): 2'-deoxy-2'-fluorocytidine
  modified_base (10)..(10): 2'-methoxyuridine
  modified_base (11)..(11): 2'-deoxy-2'-fluoroguanosine
  modified_base (12)..(12): 2'-methoxyguanosine
  modified_base (13)..(13): 2'-deoxy-2'-fluorouridine
  modified_base (14)..(14): 2'-methoxycytidine
  modified_base (15)..(15): 2'-deoxy-2'-fluorouridine
  modified_base (16)..(16): 2'-deoxy-2'-fluorouridine
  modified_base (17)..(17): 2'-methoxyuridine
  modified_base (18)..(18): 2'-deoxy-2'-fluorocytidine
  modified_base (19)..(19): 2'-methoxyuridine
  modified_base (20)..(20): 2'-deoxy-2'-fluoroadenosine
  modified_base (21)..(21): 2'-methoxyuridine
  modified_base (22)..(22): 2'-deoxy-2'-fluoroadenosine
  modified_base (23)..(23): 2'-methoxyuridine
  misc_feature (23)..(24): 5'-phosphorothioated
  modified_base (24)..(24): 2'-deoxy-2'-fluorocytidine
  misc_feature (24)..(25): 5'-phosphorothioated
  modified_base (25)..(25): 2'-methoxyuridine
agcaaggacuggucuuucuauaucu

SEQ ID NO: 71 - DNA, 55 bp, Artificial Sequence
  RT primer
gtcgtatccagtgcagggtccgaggtattcgcactggatacgactcctatgtctg

SEQ ID NO: 72 - DNA, 21 bp, Artificial Sequence
  forward primer
cgcgcgcgataaaatctacag

SEQ ID NO: 73 - DNA, 16 bp, Artificial Sequence
  reverse primer
gtgcagggtccgaggt

SEQ ID NO: 74 - DNA, 16 bp, Artificial Sequence
  TaqMan probe
ctggatacgactccta